European Patent Application EP 4 679 090 A1, published January 14, 2026. Title: A TARGET-DIRECTED AND CRL-AGNOSTIC PROXIMITY ASSAY. Applicant: Proxygen GmbH. Application EP. The sequence listing filed with the application follows.

SEQUENCE LISTING (44 sequences)

SEQ ID NO: 1 - DNA, 5496 bp, synthetic construct
  source 1..5496: mol_type = other DNA
cgttacataacttacggtaaatggcccgcctggctgaccgcccaacgacccccgcccattgacgtcaataatgacgtatgttcccatagtaacgccaatagggactttccattgacgtcaatgggtggagtatttacggtaaactgcccacttggcagtacatcaagtgtatcatatgccaagtacgccccctattgacgtcaatgacggtaaatggcccgcctggcattatgcccagtacatgaccttatgggactttcctacttggcagtacatctacgtattagtcatcgctattaccatgctgatgcggttttggcagtacatcaatgggcgtggatagcggtttgactcacggggatttccaagtctccaccccattgacgtcaatgggagtttgttttggcaccaaaatcaacgggactttccaaaatgtcgtaacaactccgccccattgacgcaaatgggcggtaggcgtgtacggtgggaggtctatataagcagagctggtttagtgaaccgtcagatcagatctttgtcgatcctaccatccactcgacacacccgccagcggccgcgccaccatgtatccgtatgacgtcccggactatgcaggatcctatccatatgacgttccagattacgctatggcagaaatcggtactggctttccattcgacccccattatgtggaagtcctgggcgagcgcatgcactacgtcgatgttggtccgcgcgatggcacccctgtgctgttcctgcacggtaacccgacctcctcctacgtgtggcgcaacatcatcccgcatgttgcaccgacccatcgctgcattgctccagacctgatcggtatgggcaaatccgacaaaccagacctgggttatttcttcgacgaccacgtccgcttcatggatgccttcatcgaagccctgggtctggaagaggtcgtcctggtcattcacgactggggctccgctctgggtttccactgggccaagcgcaatccagagcgcgtcaaaggtattgcatttatggagttcatccgccctatcccgacctgggacgaatggccagaatttgcccgcgagaccttccaggccttccgcaccaccgacgtcggccgcaagctgatcatcgatcagaacgtttttatcgagggtacgctgccgatgggtgtcgtccgcccgctgactgaagtcgagatggaccattaccgcgagccgttcctgaatcctgttgaccgcgagccactgtggcgcttcccaaacgagctgccaatcgccggtgagccagcgaacatcgtcgcgctggtcgaagaatacatggactggctgcaccagtcccctgtcccgaagctgctgttctggggcaccccaggcgttctgatcccaccggccgaagccgctcgcctggccaaaagcctgcctaactgcaaggctgtggacatcggcccgggtctgaatctgctgcaagaagacaacccggacctgatcggcagcgagatcgcgcgctggctgtcgacgctcgagatttccggcggcggaggcggttctgcggcagcgatggatgtggataccccgagcggcaccaacagcggcgcgggcaagaagcgctttgaagtgaaaaagtggaatgcagtagccctctgggcctgggatattgtggttgataactgtgccatctgcaggaaccacattatggatctttgcatagaatgtcaagctaaccaggcgtccgctacttcagaagagtgtactgtcgcatggggagtctgtaaccatgcttttcacttccactgcatctctcgctggctcaaaacacgacaggtgtgtccattggacaacagagagtgggaattccaaaagtatgggcactagggatccgcaggcctctgctagcttgactgactgagatacagcgtaccttcagctcacagacatgataagatacattgatgagtttggacaaaccacaactagaatgcagtgaaaaaaatgctttatttgtgaaatttgtgatgctattgctttatttgtaaccattataagctgcaataaacaagttaacaacaacaattgcattcattttatgtttcaggttcagggggaggtgtgggaggttttttaaagcaagtaaaacctctacaaatgtggtattggcccatctctatcggtatcgtagcataaccccttggggcctctaaacgggtcttgaggggttttttgtgcccctcgggccggattgctatctaccggcattggcgcagaaaaaaatgcctgatgcgacgctgcgcgtcttatactcccacatatgccagattcagcaacggatacggcttccccaacttgcccacttccatacgtgtcctccttaccagaaatttatccttaaggtcgtcagctatcctgcaggcgatctctcgatttcgatcaagacattcctttaatggtcttttctggacaccactaggggtcagaagtagttcatcaaactttcttccctccctaatctcattggttaccttgggctatcgaaacttaattaaccagtcaagtcagctacttggcgagatcgacttgtctgggtttcgactacgctcagaattgcgtcagtcaagttcgatctggtccttgctattgcacccgttctccgattacgagtttcatttaaatcatgtgagcaaaaggccagcaaaaggccaggaaccgtaaaaaggccgcgttgctggcgtttttccataggctccgcccccctgacgagcatcacaaaaatcgacgctcaagtcagaggtggcgaaacccgacaggactataaagataccaggcgtttccccctggaagctccctcgtgcgctctcctgttccgaccctgccgcttaccggatacctgtccgcctttctcccttcgggaagcgtggcgctttctcatagctcacgctgtaggtatctcagttcggtgtaggtcgttcgctccaagctgggctgtgtgcacgaaccccccgttcagcccgaccgctgcgccttatccggtaactatcgtcttgagtccaacccggtaagacacgacttatcgccactggcagcagccactggtaacaggattagcagagcgaggtatgtaggcggtgctacagagttcttgaagtggtggcctaactacggctacactagaagaacagtatttggtatctgcgctctgctgaagccagttaccttcggaaaaagagttggtagctcttgatccggcaaacaaaccaccgctggtagcggtggtttttttgtttgcaagcagcagattacgcgcagaaaaaaaggatctcaagaagatcctttgatcttttctacggggtctgacgctcagtggaacgaaaactcacgttaagggattttggtcatgagattatcaaaaaggatcttcacctagatccttttaaattaaaaatgaagttttaaatcaatctaaagtatatatgagtaaacttggtctgacagttaccaatgcttaatcagtgaggcacctatctcagcgatctgtctatttcgttcatccatagttgcatttaaatttccgaactctccaaggccctcgtcggaaaatcttcaaacctttcgtccgatccatcttgcaggctacctctcgaacgaactatcgcaagtctcttggccggccttgcgccttggctattgcttggcagcgcctatcgccaggtattactccaatcccgaatatccgagatcgggatcacccgagagaagttcaacctacatcctcaatcccgatctatccgagatccgaggaatatcgaaatcggggcgcgcctggtgtaccgagaacgatcctctcagtgcgagtctcgacgatccatatcgttgcttggcagtcagccagtcggaatccagcttgggacccaggaagtccaatcgtcagatattgtactcaagcctggtcacggcagcgtaccgatctgtttaaacctagatattgatagtctgatcggtcaacgtataatcgagtcctagcttttgcaaacatctatcaagagacaggatcagcaggaggctttcgcatgagtattcaacatttccgtgtcgcccttattcccttttttgcggcattttgccttcctgtttttgctcacccagaaacgctggtgaaagtaaaagatgctgaagatcagttgggtgcgcgagtgggttacatcgaactggatctcaacagcggtaagatccttgagagttttcgccccgaagaacgctttccaatgatgagcacttttaaagttctgctatgtggcgcggtattatcccgtattgacgccgggcaagagcaactcggtcgccgcatacactattctcagaatgacttggttgagtattcaccagtcacagaaaagcatcttacggatggcatgacagtaagagaattatgcagtgctgccataaccatgagtgataacactgcggccaacttacttctgacaacgattggaggaccgaaggagctaaccgcttttttgcacaacatgggggatcatgtaactcgccttgatcgttgggaaccggagctgaatgaagccataccaaacgacgagcgtgacaccacgatgcctgtagcaatggcaacaaccttgcgtaaactattaactggcgaactacttactctagcttcccggcaacagttgatagactggatggaggcggataaagttgcaggaccacttctgcgctcggcccttccggctggctggtttattgctgataaatctggagccggtgagcgtgggtctcgcggtatcattgcagcactggggccagatggtaagccctcccgtatcgtagttatctacacgacggggagtcaggcaactatggatgaacgaaatagacagatcgctgagataggtgcctcactgattaagcattggtaaccgattctaggtgcattggcgcagaaaaaaatgcctgatgcgacgctgcgcgtcttatactcccacatatgccagattcagcaacggatacggcttccccaacttgcccacttccatacgtgtcctccttaccagaaatttatccttaagatcccgaatcgtttaaactcgactctggctctatcgaatctccgtcgtttcgagcttacgcgaacagccgtggcgctcatttgctcgtcgggcatcgaatctcgtcagctatcgtcagcttacctttttggcagcgatcgcggctcccgacatcttggaccattagctccacaggtatcttcttccctctagtggtcataacagcagcttcagctacctctcaattcaaaaaacccctcaagacccgtttagaggccccaaggggttatgctatcaatcgttgcgttacacacacaaaaaaccaacacacatccatcttcgatggatagcgattttattatctaactgctgatcgagtgtagccagatctagtaatcaattacggggtcattagttcatagcccatatatggagttccg

SEQ ID NO: 2 - DNA, 5493 bp, synthetic construct
  source 1..5493: mol_type = other DNA
gccaccatggcggcagcgatggatgtggataccccgagcggcaccaacagcggcgcgggcaagaagcgctttgaagtgaaaaagtggaatgcagtagccctctgggcctgggatattgtggttgataactgtgccatctgcaggaaccacattatggatctttgcatagaatgtcaagctaaccaggcgtccgctacttcagaagagtgtactgtcgcatggggagtctgtaaccatgcttttcacttccactgcatctctcgctggctcaaaacacgacaggtgtgtccattggacaacagagagtgggaattccaaaagtatgggcacggcggaggcggttctgcagaaatcggtactggctttccattcgacccccattatgtggaagtcctgggcgagcgcatgcactacgtcgatgttggtccgcgcgatggcacccctgtgctgttcctgcacggtaacccgacctcctcctacgtgtggcgcaacatcatcccgcatgttgcaccgacccatcgctgcattgctccagacctgatcggtatgggcaaatccgacaaaccagacctgggttatttcttcgacgaccacgtccgcttcatggatgccttcatcgaagccctgggtctggaagaggtcgtcctggtcattcacgactggggctccgctctgggtttccactgggccaagcgcaatccagagcgcgtcaaaggtattgcatttatggagttcatccgccctatcccgacctgggacgaatggccagaatttgcccgcgagaccttccaggccttccgcaccaccgacgtcggccgcaagctgatcatcgatcagaacgtttttatcgagggtacgctgccgatgggtgtcgtccgcccgctgactgaagtcgagatggaccattaccgcgagccgttcctgaatcctgttgaccgcgagccactgtggcgcttcccaaacgagctgccaatcgccggtgagccagcgaacatcgtcgcgctggtcgaagaatacatggactggctgcaccagtcccctgtcccgaagctgctgttctggggcaccccaggcgttctgatcccaccggccgaagccgctcgcctggccaaaagcctgcctaactgcaaggctgtggacatcggcccgggtctgaatctgctgcaagaagacaacccggacctgatcggcagcgagatcgcgcgctggctgtcgacgctcgagatttccggctatccgtatgacgtcccggactatgcaggatcctatccatatgacgttccagattacgcttaaggatccgcaggcctctgctagcttgactgactgagatacagcgtaccttcagctcacagacatgataagatacattgatgagtttggacaaaccacaactagaatgcagtgaaaaaaatgctttatttgtgaaatttgtgatgctattgctttatttgtaaccattataagctgcaataaacaagttaacaacaacaattgcattcattttatgtttcaggttcagggggaggtgtgggaggttttttaaagcaagtaaaacctctacaaatgtggtattggcccatctctatcggtatcgtagcataaccccttggggcctctaaacgggtcttgaggggttttttgtgcccctcgggccggattgctatctaccggcattggcgcagaaaaaaatgcctgatgcgacgctgcgcgtcttatactcccacatatgccagattcagcaacggatacggcttccccaacttgcccacttccatacgtgtcctccttaccagaaatttatccttaaggtcgtcagctatcctgcaggcgatctctcgatttcgatcaagacattcctttaatggtcttttctggacaccactaggggtcagaagtagttcatcaaactttcttccctccctaatctcattggttaccttgggctatcgaaacttaattaaccagtcaagtcagctacttggcgagatcgacttgtctgggtttcgactacgctcagaattgcgtcagtcaagttcgatctggtccttgctattgcacccgttctccgattacgagtttcatttaaatcatgtgagcaaaaggccagcaaaaggccaggaaccgtaaaaaggccgcgttgctggcgtttttccataggctccgcccccctgacgagcatcacaaaaatcgacgctcaagtcagaggtggcgaaacccgacaggactataaagataccaggcgtttccccctggaagctccctcgtgcgctctcctgttccgaccctgccgcttaccggatacctgtccgcctttctcccttcgggaagcgtggcgctttctcatagctcacgctgtaggtatctcagttcggtgtaggtcgttcgctccaagctgggctgtgtgcacgaaccccccgttcagcccgaccgctgcgccttatccggtaactatcgtcttgagtccaacccggtaagacacgacttatcgccactggcagcagccactggtaacaggattagcagagcgaggtatgtaggcggtgctacagagttcttgaagtggtggcctaactacggctacactagaagaacagtatttggtatctgcgctctgctgaagccagttaccttcggaaaaagagttggtagctcttgatccggcaaacaaaccaccgctggtagcggtggtttttttgtttgcaagcagcagattacgcgcagaaaaaaaggatctcaagaagatcctttgatcttttctacggggtctgacgctcagtggaacgaaaactcacgttaagggattttggtcatgagattatcaaaaaggatcttcacctagatccttttaaattaaaaatgaagttttaaatcaatctaaagtatatatgagtaaacttggtctgacagttaccaatgcttaatcagtgaggcacctatctcagcgatctgtctatttcgttcatccatagttgcatttaaatttccgaactctccaaggccctcgtcggaaaatcttcaaacctttcgtccgatccatcttgcaggctacctctcgaacgaactatcgcaagtctcttggccggccttgcgccttggctattgcttggcagcgcctatcgccaggtattactccaatcccgaatatccgagatcgggatcacccgagagaagttcaacctacatcctcaatcccgatctatccgagatccgaggaatatcgaaatcggggcgcgcctggtgtaccgagaacgatcctctcagtgcgagtctcgacgatccatatcgttgcttggcagtcagccagtcggaatccagcttgggacccaggaagtccaatcgtcagatattgtactcaagcctggtcacggcagcgtaccgatctgtttaaacctagatattgatagtctgatcggtcaacgtataatcgagtcctagcttttgcaaacatctatcaagagacaggatcagcaggaggctttcgcatgagtattcaacatttccgtgtcgcccttattcccttttttgcggcattttgccttcctgtttttgctcacccagaaacgctggtgaaagtaaaagatgctgaagatcagttgggtgcgcgagtgggttacatcgaactggatctcaacagcggtaagatccttgagagttttcgccccgaagaacgctttccaatgatgagcacttttaaagttctgctatgtggcgcggtattatcccgtattgacgccgggcaagagcaactcggtcgccgcatacactattctcagaatgacttggttgagtattcaccagtcacagaaaagcatcttacggatggcatgacagtaagagaattatgcagtgctgccataaccatgagtgataacactgcggccaacttacttctgacaacgattggaggaccgaaggagctaaccgcttttttgcacaacatgggggatcatgtaactcgccttgatcgttgggaaccggagctgaatgaagccataccaaacgacgagcgtgacaccacgatgcctgtagcaatggcaacaaccttgcgtaaactattaactggcgaactacttactctagcttcccggcaacagttgatagactggatggaggcggataaagttgcaggaccacttctgcgctcggcccttccggctggctggtttattgctgataaatctggagccggtgagcgtgggtctcgcggtatcattgcagcactggggccagatggtaagccctcccgtatcgtagttatctacacgacggggagtcaggcaactatggatgaacgaaatagacagatcgctgagataggtgcctcactgattaagcattggtaaccgattctaggtgcattggcgcagaaaaaaatgcctgatgcgacgctgcgcgtcttatactcccacatatgccagattcagcaacggatacggcttccccaacttgcccacttccatacgtgtcctccttaccagaaatttatccttaagatcccgaatcgtttaaactcgactctggctctatcgaatctccgtcgtttcgagcttacgcgaacagccgtggcgctcatttgctcgtcgggcatcgaatctcgtcagctatcgtcagcttacctttttggcagcgatcgcggctcccgacatcttggaccattagctccacaggtatcttcttccctctagtggtcataacagcagcttcagctacctctcaattcaaaaaacccctcaagacccgtttagaggccccaaggggttatgctatcaatcgttgcgttacacacacaaaaaaccaacacacatccatcttcgatggatagcgattttattatctaactgctgatcgagtgtagccagatctagtaatcaattacggggtcattagttcatagcccatatatggagttccgcgttacataacttacggtaaatggcccgcctggctgaccgcccaacgacccccgcccattgacgtcaataatgacgtatgttcccatagtaacgccaatagggactttccattgacgtcaatgggtggagtatttacggtaaactgcccacttggcagtacatcaagtgtatcatatgccaagtacgccccctattgacgtcaatgacggtaaatggcccgcctggcattatgcccagtacatgaccttatgggactttcctacttggcagtacatctacgtattagtcatcgctattaccatgctgatgcggttttggcagtacatcaatgggcgtggatagcggtttgactcacggggatttccaagtctccaccccattgacgtcaatgggagtttgttttggcaccaaaatcaacgggactttccaaaatgtcgtaacaactccgccccattgacgcaaatgggcggtaggcgtgtacggtgggaggtctatataagcagagctggtttagtgaaccgtcagatcagatctttgtcgatcctaccatccactcgacacacccgccagcggccgc

SEQ ID NO: 3 - DNA, 5526 bp, synthetic construct
  source 1..5526: mol_type = other DNA
gccaccatgtatccgtatgacgtcccggactatgcaggatcctatccatatgacgttccagattacgctatggcagaaatcggtactggctttccattcgacccccattatgtggaagtcctgggcgagcgcatgcactacgtcgatgttggtccgcgcgatggcacccctgtgctgttcctgcacggtaacccgacctcctcctacgtgtggcgcaacatcatcccgcatgttgcaccgacccatcgctgcattgctccagacctgatcggtatgggcaaatccgacaaaccagacctgggttatttcttcgacgaccacgtccgcttcatggatgccttcatcgaagccctgggtctggaagaggtcgtcctggtcattcacgactggggctccgctctgggtttccactgggccaagcgcaatccagagcgcgtcaaaggtattgcatttatggagttcatccgccctatcccgacctgggacgaatggccagaatttgcccgcgagaccttccaggccttccgcaccaccgacgtcggccgcaagctgatcatcgatcagaacgtttttatcgagggtacgctgccgatgggtgtcgtccgcccgctgactgaagtcgagatggaccattaccgcgagccgttcctgaatcctgttgaccgcgagccactgtggcgcttcccaaacgagctgccaatcgccggtgagccagcgaacatcgtcgcgctggtcgaagaatacatggactggctgcaccagtcccctgtcccgaagctgctgttctggggcaccccaggcgttctgatcccaccggccgaagccgctcgcctggccaaaagcctgcctaactgcaaggctgtggacatcggcccgggtctgaatctgctgcaagaagacaacccggacctgatcggcagcgagatcgcgcgctggctgtcgacgctcgagatttccggcggcggaggcggttctggtggcggaggttctgggggtggcggatctgcggcagcgatggatgtggataccccgagcggcaccaacagcggcgcgggcaagaagcgctttgaagtgaaaaagtggaatgcagtagccctctgggcctgggatattgtggttgataactgtgccatctgcaggaaccacattatggatctttgcatagaatgtcaagctaaccaggcgtccgctacttcagaagagtgtactgtcgcatggggagtctgtaaccatgcttttcacttccactgcatctctcgctggctcaaaacacgacaggtgtgtccattggacaacagagagtgggaattccaaaagtatgggcactagggatccgcaggcctctgctagcttgactgactgagatacagcgtaccttcagctcacagacatgataagatacattgatgagtttggacaaaccacaactagaatgcagtgaaaaaaatgctttatttgtgaaatttgtgatgctattgctttatttgtaaccattataagctgcaataaacaagttaacaacaacaattgcattcattttatgtttcaggttcagggggaggtgtgggaggttttttaaagcaagtaaaacctctacaaatgtggtattggcccatctctatcggtatcgtagcataaccccttggggcctctaaacgggtcttgaggggttttttgtgcccctcgggccggattgctatctaccggcattggcgcagaaaaaaatgcctgatgcgacgctgcgcgtcttatactcccacatatgccagattcagcaacggatacggcttccccaacttgcccacttccatacgtgtcctccttaccagaaatttatccttaaggtcgtcagctatcctgcaggcgatctctcgatttcgatcaagacattcctttaatggtcttttctggacaccactaggggtcagaagtagttcatcaaactttcttccctccctaatctcattggttaccttgggctatcgaaacttaattaaccagtcaagtcagctacttggcgagatcgacttgtctgggtttcgactacgctcagaattgcgtcagtcaagttcgatctggtccttgctattgcacccgttctccgattacgagtttcatttaaatcatgtgagcaaaaggccagcaaaaggccaggaaccgtaaaaaggccgcgttgctggcgtttttccataggctccgcccccctgacgagcatcacaaaaatcgacgctcaagtcagaggtggcgaaacccgacaggactataaagataccaggcgtttccccctggaagctccctcgtgcgctctcctgttccgaccctgccgcttaccggatacctgtccgcctttctcccttcgggaagcgtggcgctttctcatagctcacgctgtaggtatctcagttcggtgtaggtcgttcgctccaagctgggctgtgtgcacgaaccccccgttcagcccgaccgctgcgccttatccggtaactatcgtcttgagtccaacccggtaagacacgacttatcgccactggcagcagccactggtaacaggattagcagagcgaggtatgtaggcggtgctacagagttcttgaagtggtggcctaactacggctacactagaagaacagtatttggtatctgcgctctgctgaagccagttaccttcggaaaaagagttggtagctcttgatccggcaaacaaaccaccgctggtagcggtggtttttttgtttgcaagcagcagattacgcgcagaaaaaaaggatctcaagaagatcctttgatcttttctacggggtctgacgctcagtggaacgaaaactcacgttaagggattttggtcatgagattatcaaaaaggatcttcacctagatccttttaaattaaaaatgaagttttaaatcaatctaaagtatatatgagtaaacttggtctgacagttaccaatgcttaatcagtgaggcacctatctcagcgatctgtctatttcgttcatccatagttgcatttaaatttccgaactctccaaggccctcgtcggaaaatcttcaaacctttcgtccgatccatcttgcaggctacctctcgaacgaactatcgcaagtctcttggccggccttgcgccttggctattgcttggcagcgcctatcgccaggtattactccaatcccgaatatccgagatcgggatcacccgagagaagttcaacctacatcctcaatcccgatctatccgagatccgaggaatatcgaaatcggggcgcgcctggtgtaccgagaacgatcctctcagtgcgagtctcgacgatccatatcgttgcttggcagtcagccagtcggaatccagcttgggacccaggaagtccaatcgtcagatattgtactcaagcctggtcacggcagcgtaccgatctgtttaaacctagatattgatagtctgatcggtcaacgtataatcgagtcctagcttttgcaaacatctatcaagagacaggatcagcaggaggctttcgcatgagtattcaacatttccgtgtcgcccttattcccttttttgcggcattttgccttcctgtttttgctcacccagaaacgctggtgaaagtaaaagatgctgaagatcagttgggtgcgcgagtgggttacatcgaactggatctcaacagcggtaagatccttgagagttttcgccccgaagaacgctttccaatgatgagcacttttaaagttctgctatgtggcgcggtattatcccgtattgacgccgggcaagagcaactcggtcgccgcatacactattctcagaatgacttggttgagtattcaccagtcacagaaaagcatcttacggatggcatgacagtaagagaattatgcagtgctgccataaccatgagtgataacactgcggccaacttacttctgacaacgattggaggaccgaaggagctaaccgcttttttgcacaacatgggggatcatgtaactcgccttgatcgttgggaaccggagctgaatgaagccataccaaacgacgagcgtgacaccacgatgcctgtagcaatggcaacaaccttgcgtaaactattaactggcgaactacttactctagcttcccggcaacagttgatagactggatggaggcggataaagttgcaggaccacttctgcgctcggcccttccggctggctggtttattgctgataaatctggagccggtgagcgtgggtctcgcggtatcattgcagcactggggccagatggtaagccctcccgtatcgtagttatctacacgacggggagtcaggcaactatggatgaacgaaatagacagatcgctgagataggtgcctcactgattaagcattggtaaccgattctaggtgcattggcgcagaaaaaaatgcctgatgcgacgctgcgcgtcttatactcccacatatgccagattcagcaacggatacggcttccccaacttgcccacttccatacgtgtcctccttaccagaaatttatccttaagatcccgaatcgtttaaactcgactctggctctatcgaatctccgtcgtttcgagcttacgcgaacagccgtggcgctcatttgctcgtcgggcatcgaatctcgtcagctatcgtcagcttacctttttggcagcgatcgcggctcccgacatcttggaccattagctccacaggtatcttcttccctctagtggtcataacagcagcttcagctacctctcaattcaaaaaacccctcaagacccgtttagaggccccaaggggttatgctatcaatcgttgcgttacacacacaaaaaaccaacacacatccatcttcgatggatagcgattttattatctaactgctgatcgagtgtagccagatctagtaatcaattacggggtcattagttcatagcccatatatggagttccgcgttacataacttacggtaaatggcccgcctggctgaccgcccaacgacccccgcccattgacgtcaataatgacgtatgttcccatagtaacgccaatagggactttccattgacgtcaatgggtggagtatttacggtaaactgcccacttggcagtacatcaagtgtatcatatgccaagtacgccccctattgacgtcaatgacggtaaatggcccgcctggcattatgcccagtacatgaccttatgggactttcctacttggcagtacatctacgtattagtcatcgctattaccatgctgatgcggttttggcagtacatcaatgggcgtggatagcggtttgactcacggggatttccaagtctccaccccattgacgtcaatgggagtttgttttggcaccaaaatcaacgggactttccaaaatgtcgtaacaactccgccccattgacgcaaatgggcggtaggcgtgtacggtgggaggtctatataagcagagctggtttagtgaaccgtcagatcagatctttgtcgatcctaccatccactcgacacacccgccagcggccgc

SEQ ID NO: 4 - DNA, 5523 bp, synthetic construct
  source 1..5523: mol_type = other DNA
gccaccatggcggcagcgatggatgtggataccccgagcggcaccaacagcggcgcgggcaagaagcgctttgaagtgaaaaagtggaatgcagtagccctctgggcctgggatattgtggttgataactgtgccatctgcaggaaccacattatggatctttgcatagaatgtcaagctaaccaggcgtccgctacttcagaagagtgtactgtcgcatggggagtctgtaaccatgcttttcacttccactgcatctctcgctggctcaaaacacgacaggtgtgtccattggacaacagagagtgggaattccaaaagtatgggcacggcggaggcggttctggtggcggaggttctgggggtggcggatctgcagaaatcggtactggctttccattcgacccccattatgtggaagtcctgggcgagcgcatgcactacgtcgatgttggtccgcgcgatggcacccctgtgctgttcctgcacggtaacccgacctcctcctacgtgtggcgcaacatcatcccgcatgttgcaccgacccatcgctgcattgctccagacctgatcggtatgggcaaatccgacaaaccagacctgggttatttcttcgacgaccacgtccgcttcatggatgccttcatcgaagccctgggtctggaagaggtcgtcctggtcattcacgactggggctccgctctgggtttccactgggccaagcgcaatccagagcgcgtcaaaggtattgcatttatggagttcatccgccctatcccgacctgggacgaatggccagaatttgcccgcgagaccttccaggccttccgcaccaccgacgtcggccgcaagctgatcatcgatcagaacgtttttatcgagggtacgctgccgatgggtgtcgtccgcccgctgactgaagtcgagatggaccattaccgcgagccgttcctgaatcctgttgaccgcgagccactgtggcgcttcccaaacgagctgccaatcgccggtgagccagcgaacatcgtcgcgctggtcgaagaatacatggactggctgcaccagtcccctgtcccgaagctgctgttctggggcaccccaggcgttctgatcccaccggccgaagccgctcgcctggccaaaagcctgcctaactgcaaggctgtggacatcggcccgggtctgaatctgctgcaagaagacaacccggacctgatcggcagcgagatcgcgcgctggctgtcgacgctcgagatttccggctatccgtatgacgtcccggactatgcaggatcctatccatatgacgttccagattacgcttaaggatccgcaggcctctgctagcttgactgactgagatacagcgtaccttcagctcacagacatgataagatacattgatgagtttggacaaaccacaactagaatgcagtgaaaaaaatgctttatttgtgaaatttgtgatgctattgctttatttgtaaccattataagctgcaataaacaagttaacaacaacaattgcattcattttatgtttcaggttcagggggaggtgtgggaggttttttaaagcaagtaaaacctctacaaatgtggtattggcccatctctatcggtatcgtagcataaccccttggggcctctaaacgggtcttgaggggttttttgtgcccctcgggccggattgctatctaccggcattggcgcagaaaaaaatgcctgatgcgacgctgcgcgtcttatactcccacatatgccagattcagcaacggatacggcttccccaacttgcccacttccatacgtgtcctccttaccagaaatttatccttaaggtcgtcagctatcctgcaggcgatctctcgatttcgatcaagacattcctttaatggtcttttctggacaccactaggggtcagaagtagttcatcaaactttcttccctccctaatctcattggttaccttgggctatcgaaacttaattaaccagtcaagtcagctacttggcgagatcgacttgtctgggtttcgactacgctcagaattgcgtcagtcaagttcgatctggtccttgctattgcacccgttctccgattacgagtttcatttaaatcatgtgagcaaaaggccagcaaaaggccaggaaccgtaaaaaggccgcgttgctggcgtttttccataggctccgcccccctgacgagcatcacaaaaatcgacgctcaagtcagaggtggcgaaacccgacaggactataaagataccaggcgtttccccctggaagctccctcgtgcgctctcctgttccgaccctgccgcttaccggatacctgtccgcctttctcccttcgggaagcgtggcgctttctcatagctcacgctgtaggtatctcagttcggtgtaggtcgttcgctccaagctgggctgtgtgcacgaaccccccgttcagcccgaccgctgcgccttatccggtaactatcgtcttgagtccaacccggtaagacacgacttatcgccactggcagcagccactggtaacaggattagcagagcgaggtatgtaggcggtgctacagagttcttgaagtggtggcctaactacggctacactagaagaacagtatttggtatctgcgctctgctgaagccagttaccttcggaaaaagagttggtagctcttgatccggcaaacaaaccaccgctggtagcggtggtttttttgtttgcaagcagcagattacgcgcagaaaaaaaggatctcaagaagatcctttgatcttttctacggggtctgacgctcagtggaacgaaaactcacgttaagggattttggtcatgagattatcaaaaaggatcttcacctagatccttttaaattaaaaatgaagttttaaatcaatctaaagtatatatgagtaaacttggtctgacagttaccaatgcttaatcagtgaggcacctatctcagcgatctgtctatttcgttcatccatagttgcatttaaatttccgaactctccaaggccctcgtcggaaaatcttcaaacctttcgtccgatccatcttgcaggctacctctcgaacgaactatcgcaagtctcttggccggccttgcgccttggctattgcttggcagcgcctatcgccaggtattactccaatcccgaatatccgagatcgggatcacccgagagaagttcaacctacatcctcaatcccgatctatccgagatccgaggaatatcgaaatcggggcgcgcctggtgtaccgagaacgatcctctcagtgcgagtctcgacgatccatatcgttgcttggcagtcagccagtcggaatccagcttgggacccaggaagtccaatcgtcagatattgtactcaagcctggtcacggcagcgtaccgatctgtttaaacctagatattgatagtctgatcggtcaacgtataatcgagtcctagcttttgcaaacatctatcaagagacaggatcagcaggaggctttcgcatgagtattcaacatttccgtgtcgcccttattcccttttttgcggcattttgccttcctgtttttgctcacccagaaacgctggtgaaagtaaaagatgctgaagatcagttgggtgcgcgagtgggttacatcgaactggatctcaacagcggtaagatccttgagagttttcgccccgaagaacgctttccaatgatgagcacttttaaagttctgctatgtggcgcggtattatcccgtattgacgccgggcaagagcaactcggtcgccgcatacactattctcagaatgacttggttgagtattcaccagtcacagaaaagcatcttacggatggcatgacagtaagagaattatgcagtgctgccataaccatgagtgataacactgcggccaacttacttctgacaacgattggaggaccgaaggagctaaccgcttttttgcacaacatgggggatcatgtaactcgccttgatcgttgggaaccggagctgaatgaagccataccaaacgacgagcgtgacaccacgatgcctgtagcaatggcaacaaccttgcgtaaactattaactggcgaactacttactctagcttcccggcaacagttgatagactggatggaggcggataaagttgcaggaccacttctgcgctcggcccttccggctggctggtttattgctgataaatctggagccggtgagcgtgggtctcgcggtatcattgcagcactggggccagatggtaagccctcccgtatcgtagttatctacacgacggggagtcaggcaactatggatgaacgaaatagacagatcgctgagataggtgcctcactgattaagcattggtaaccgattctaggtgcattggcgcagaaaaaaatgcctgatgcgacgctgcgcgtcttatactcccacatatgccagattcagcaacggatacggcttccccaacttgcccacttccatacgtgtcctccttaccagaaatttatccttaagatcccgaatcgtttaaactcgactctggctctatcgaatctccgtcgtttcgagcttacgcgaacagccgtggcgctcatttgctcgtcgggcatcgaatctcgtcagctatcgtcagcttacctttttggcagcgatcgcggctcccgacatcttggaccattagctccacaggtatcttcttccctctagtggtcataacagcagcttcagctacctctcaattcaaaaaacccctcaagacccgtttagaggccccaaggggttatgctatcaatcgttgcgttacacacacaaaaaaccaacacacatccatcttcgatggatagcgattttattatctaactgctgatcgagtgtagccagatctagtaatcaattacggggtcattagttcatagcccatatatggagttccgcgttacataacttacggtaaatggcccgcctggctgaccgcccaacgacccccgcccattgacgtcaataatgacgtatgttcccatagtaacgccaatagggactttccattgacgtcaatgggtggagtatttacggtaaactgcccacttggcagtacatcaagtgtatcatatgccaagtacgccccctattgacgtcaatgacggtaaatggcccgcctggcattatgcccagtacatgaccttatgggactttcctacttggcagtacatctacgtattagtcatcgctattaccatgctgatgcggttttggcagtacatcaatgggcgtggatagcggtttgactcacggggatttccaagtctccaccccattgacgtcaatgggagtttgttttggcaccaaaatcaacgggactttccaaaatgtcgtaacaactccgccccattgacgcaaatgggcggtaggcgtgtacggtgggaggtctatataagcagagctggtttagtgaaccgtcagatcagatctttgtcgatcctaccatccactcgacacacccgccagcggccgc

SEQ ID NO: 5 - DNA, 5118 bp, synthetic construct
  source 1..5118: mol_type = other DNA
gccaccatgtatccgtatgacgtcccggactatgcaggatcctatccatatgacgttccagattacgctatggtcttcacactcgaagatttcgttggggactggcgacagacagccggctacaacctggaccaagtccttgaacagggaggtgtgtccagtttgtttcagaatctcggggtgtccgtaactccgatccaaaggattgtcctgagcggtgaaaatgggctgaagatcgacatccatgtcatcatcccgtatgaaggtctgagcggcgaccaaatgggccagatcgaaaaaatttttaaggtggtgtaccctgtggatgatcatcactttaaggtgatcctgcactatggcacactggtaatcgacggggttacgccgaacatgatcgactatttcggacggccgtatgaaggcatcgccgtgttcgacggcaaaaagatcactgtaacagggaccctgtggaacggcaacaaaattatcgacgagcgcctgatcaaccccgacggctccctgctgttccgagtaaccatcaacggagtgaccggctggcggctgtgcgaacgcattctggcgggcggaggcggttctgcggcagcgatggatgtggataccccgagcggcaccaacagcggcgcgggcaagaagcgctttgaagtgaaaaagtggaatgcagtagccctctgggcctgggatattgtggttgataactgtgccatctgcaggaaccacattatggatctttgcatagaatgtcaagctaaccaggcgtccgctacttcagaagagtgtactgtcgcatggggagtctgtaaccatgcttttcacttccactgcatctctcgctggctcaaaacacgacaggtgtgtccattggacaacagagagtgggaattccaaaagtatgggcactagggatccgcaggcctctgctagcttgactgactgagatacagcgtaccttcagctcacagacatgataagatacattgatgagtttggacaaaccacaactagaatgcagtgaaaaaaatgctttatttgtgaaatttgtgatgctattgctttatttgtaaccattataagctgcaataaacaagttaacaacaacaattgcattcattttatgtttcaggttcagggggaggtgtgggaggttttttaaagcaagtaaaacctctacaaatgtggtattggcccatctctatcggtatcgtagcataaccccttggggcctctaaacgggtcttgaggggttttttgtgcccctcgggccggattgctatctaccggcattggcgcagaaaaaaatgcctgatgcgacgctgcgcgtcttatactcccacatatgccagattcagcaacggatacggcttccccaacttgcccacttccatacgtgtcctccttaccagaaatttatccttaaggtcgtcagctatcctgcaggcgatctctcgatttcgatcaagacattcctttaatggtcttttctggacaccactaggggtcagaagtagttcatcaaactttcttccctccctaatctcattggttaccttgggctatcgaaacttaattaaccagtcaagtcagctacttggcgagatcgacttgtctgggtttcgactacgctcagaattgcgtcagtcaagttcgatctggtccttgctattgcacccgttctccgattacgagtttcatttaaatcatgtgagcaaaaggccagcaaaaggccaggaaccgtaaaaaggccgcgttgctggcgtttttccataggctccgcccccctgacgagcatcacaaaaatcgacgctcaagtcagaggtggcgaaacccgacaggactataaagataccaggcgtttccccctggaagctccctcgtgcgctctcctgttccgaccctgccgcttaccggatacctgtccgcctttctcccttcgggaagcgtggcgctttctcatagctcacgctgtaggtatctcagttcggtgtaggtcgttcgctccaagctgggctgtgtgcacgaaccccccgttcagcccgaccgctgcgccttatccggtaactatcgtcttgagtccaacccggtaagacacgacttatcgccactggcagcagccactggtaacaggattagcagagcgaggtatgtaggcggtgctacagagttcttgaagtggtggcctaactacggctacactagaagaacagtatttggtatctgcgctctgctgaagccagttaccttcggaaaaagagttggtagctcttgatccggcaaacaaaccaccgctggtagcggtggtttttttgtttgcaagcagcagattacgcgcagaaaaaaaggatctcaagaagatcctttgatcttttctacggggtctgacgctcagtggaacgaaaactcacgttaagggattttggtcatgagattatcaaaaaggatcttcacctagatccttttaaattaaaaatgaagttttaaatcaatctaaagtatatatgagtaaacttggtctgacagttaccaatgcttaatcagtgaggcacctatctcagcgatctgtctatttcgttcatccatagttgcatttaaatttccgaactctccaaggccctcgtcggaaaatcttcaaacctttcgtccgatccatcttgcaggctacctctcgaacgaactatcgcaagtctcttggccggccttgcgccttggctattgcttggcagcgcctatcgccaggtattactccaatcccgaatatccgagatcgggatcacccgagagaagttcaacctacatcctcaatcccgatctatccgagatccgaggaatatcgaaatcggggcgcgcctggtgtaccgagaacgatcctctcagtgcgagtctcgacgatccatatcgttgcttggcagtcagccagtcggaatccagcttgggacccaggaagtccaatcgtcagatattgtactcaagcctggtcacggcagcgtaccgatctgtttaaacctagatattgatagtctgatcggtcaacgtataatcgagtcctagcttttgcaaacatctatcaagagacaggatcagcaggaggctttcgcatgagtattcaacatttccgtgtcgcccttattcccttttttgcggcattttgccttcctgtttttgctcacccagaaacgctggtgaaagtaaaagatgctgaagatcagttgggtgcgcgagtgggttacatcgaactggatctcaacagcggtaagatccttgagagttttcgccccgaagaacgctttccaatgatgagcacttttaaagttctgctatgtggcgcggtattatcccgtattgacgccgggcaagagcaactcggtcgccgcatacactattctcagaatgacttggttgagtattcaccagtcacagaaaagcatcttacggatggcatgacagtaagagaattatgcagtgctgccataaccatgagtgataacactgcggccaacttacttctgacaacgattggaggaccgaaggagctaaccgcttttttgcacaacatgggggatcatgtaactcgccttgatcgttgggaaccggagctgaatgaagccataccaaacgacgagcgtgacaccacgatgcctgtagcaatggcaacaaccttgcgtaaactattaactggcgaactacttactctagcttcccggcaacagttgatagactggatggaggcggataaagttgcaggaccacttctgcgctcggcccttccggctggctggtttattgctgataaatctggagccggtgagcgtgggtctcgcggtatcattgcagcactggggccagatggtaagccctcccgtatcgtagttatctacacgacggggagtcaggcaactatggatgaacgaaatagacagatcgctgagataggtgcctcactgattaagcattggtaaccgattctaggtgcattggcgcagaaaaaaatgcctgatgcgacgctgcgcgtcttatactcccacatatgccagattcagcaacggatacggcttccccaacttgcccacttccatacgtgtcctccttaccagaaatttatccttaagatcccgaatcgtttaaactcgactctggctctatcgaatctccgtcgtttcgagcttacgcgaacagccgtggcgctcatttgctcgtcgggcatcgaatctcgtcagctatcgtcagcttacctttttggcagcgatcgcggctcccgacatcttggaccattagctccacaggtatcttcttccctctagtggtcataacagcagcttcagctacctctcaattcaaaaaacccctcaagacccgtttagaggccccaaggggttatgctatcaatcgttgcgttacacacacaaaaaaccaacacacatccatcttcgatggatagcgattttattatctaactgctgatcgagtgtagccagatctagtaatcaattacggggtcattagttcatagcccatatatggagttccgcgttacataacttacggtaaatggcccgcctggctgaccgcccaacgacccccgcccattgacgtcaataatgacgtatgttcccatagtaacgccaatagggactttccattgacgtcaatgggtggagtatttacggtaaactgcccacttggcagtacatcaagtgtatcatatgccaagtacgccccctattgacgtcaatgacggtaaatggcccgcctggcattatgcccagtacatgaccttatgggactttcctacttggcagtacatctacgtattagtcatcgctattaccatgctgatgcggttttggcagtacatcaatgggcgtggatagcggtttgactcacggggatttccaagtctccaccccattgacgtcaatgggagtttgttttggcaccaaaatcaacgggactttccaaaatgtcgtaacaactccgccccattgacgcaaatgggcggtaggcgtgtacggtgggaggtctatataagcagagctggtttagtgaaccgtcagatcagatctttgtcgatcctaccatccactcgacacacccgccagcggccgc

SEQ ID NO: 6 - DNA, 5115 bp, synthetic construct
  source 1..5115: mol_type = other DNA
gccaccatggcggcagcgatggatgtggataccccgagcggcaccaacagcggcgcgggcaagaagcgctttgaagtgaaaaagtggaatgcagtagccctctgggcctgggatattgtggttgataactgtgccatctgcaggaaccacattatggatctttgcatagaatgtcaagctaaccaggcgtccgctacttcagaagagtgtactgtcgcatggggagtctgtaaccatgcttttcacttccactgcatctctcgctggctcaaaacacgacaggtgtgtccattggacaacagagagtgggaattccaaaagtatgggcacggcggaggcggttctgtcttcacactcgaagatttcgttggggactggcgacagacagccggctacaacctggaccaagtccttgaacagggaggtgtgtccagtttgtttcagaatctcggggtgtccgtaactccgatccaaaggattgtcctgagcggtgaaaatgggctgaagatcgacatccatgtcatcatcccgtatgaaggtctgagcggcgaccaaatgggccagatcgaaaaaatttttaaggtggtgtaccctgtggatgatcatcactttaaggtgatcctgcactatggcacactggtaatcgacggggttacgccgaacatgatcgactatttcggacggccgtatgaaggcatcgccgtgttcgacggcaaaaagatcactgtaacagggaccctgtggaacggcaacaaaattatcgacgagcgcctgatcaaccccgacggctccctgctgttccgagtaaccatcaacggagtgaccggctggcggctgtgcgaacgcattctggcgtatccgtatgacgtcccggactatgcaggatcctatccatatgacgttccagattacgcttaaggatccgcaggcctctgctagcttgactgactgagatacagcgtaccttcagctcacagacatgataagatacattgatgagtttggacaaaccacaactagaatgcagtgaaaaaaatgctttatttgtgaaatttgtgatgctattgctttatttgtaaccattataagctgcaataaacaagttaacaacaacaattgcattcattttatgtttcaggttcagggggaggtgtgggaggttttttaaagcaagtaaaacctctacaaatgtggtattggcccatctctatcggtatcgtagcataaccccttggggcctctaaacgggtcttgaggggttttttgtgcccctcgggccggattgctatctaccggcattggcgcagaaaaaaatgcctgatgcgacgctgcgcgtcttatactcccacatatgccagattcagcaacggatacggcttccccaacttgcccacttccatacgtgtcctccttaccagaaatttatccttaaggtcgtcagctatcctgcaggcgatctctcgatttcgatcaagacattcctttaatggtcttttctggacaccactaggggtcagaagtagttcatcaaactttcttccctccctaatctcattggttaccttgggctatcgaaacttaattaaccagtcaagtcagctacttggcgagatcgacttgtctgggtttcgactacgctcagaattgcgtcagtcaagttcgatctggtccttgctattgcacccgttctccgattacgagtttcatttaaatcatgtgagcaaaaggccagcaaaaggccaggaaccgtaaaaaggccgcgttgctggcgtttttccataggctccgcccccctgacgagcatcacaaaaatcgacgctcaagtcagaggtggcgaaacccgacaggactataaagataccaggcgtttccccctggaagctccctcgtgcgctctcctgttccgaccctgccgcttaccggatacctgtccgcctttctcccttcgggaagcgtggcgctttctcatagctcacgctgtaggtatctcagttcggtgtaggtcgttcgctccaagctgggctgtgtgcacgaaccccccgttcagcccgaccgctgcgccttatccggtaactatcgtcttgagtccaacccggtaagacacgacttatcgccactggcagcagccactggtaacaggattagcagagcgaggtatgtaggcggtgctacagagttcttgaagtggtggcctaactacggctacactagaagaacagtatttggtatctgcgctctgctgaagccagttaccttcggaaaaagagttggtagctcttgatccggcaaacaaaccaccgctggtagcggtggtttttttgtttgcaagcagcagattacgcgcagaaaaaaaggatctcaagaagatcctttgatcttttctacggggtctgacgctcagtggaacgaaaactcacgttaagggattttggtcatgagattatcaaaaaggatcttcacctagatccttttaaattaaaaatgaagttttaaatcaatctaaagtatatatgagtaaacttggtctgacagttaccaatgcttaatcagtgaggcacctatctcagcgatctgtctatttcgttcatccatagttgcatttaaatttccgaactctccaaggccctcgtcggaaaatcttcaaacctttcgtccgatccatcttgcaggctacctctcgaacgaactatcgcaagtctcttggccggccttgcgccttggctattgcttggcagcgcctatcgccaggtattactccaatcccgaatatccgagatcgggatcacccgagagaagttcaacctacatcctcaatcccgatctatccgagatccgaggaatatcgaaatcggggcgcgcctggtgtaccgagaacgatcctctcagtgcgagtctcgacgatccatatcgttgcttggcagtcagccagtcggaatccagcttgggacccaggaagtccaatcgtcagatattgtactcaagcctggtcacggcagcgtaccgatctgtttaaacctagatattgatagtctgatcggtcaacgtataatcgagtcctagcttttgcaaacatctatcaagagacaggatcagcaggaggctttcgcatgagtattcaacatttccgtgtcgcccttattcccttttttgcggcattttgccttcctgtttttgctcacccagaaacgctggtgaaagtaaaagatgctgaagatcagttgggtgcgcgagtgggttacatcgaactggatctcaacagcggtaagatccttgagagttttcgccccgaagaacgctttccaatgatgagcacttttaaagttctgctatgtggcgcggtattatcccgtattgacgccgggcaagagcaactcggtcgccgcatacactattctcagaatgacttggttgagtattcaccagtcacagaaaagcatcttacggatggcatgacagtaagagaattatgcagtgctgccataaccatgagtgataacactgcggccaacttacttctgacaacgattggaggaccgaaggagctaaccgcttttttgcacaacatgggggatcatgtaactcgccttgatcgttgggaaccggagctgaatgaagccataccaaacgacgagcgtgacaccacgatgcctgtagcaatggcaacaaccttgcgtaaactattaactggcgaactacttactctagcttcccggcaacagttgatagactggatggaggcggataaagttgcaggaccacttctgcgctcggcccttccggctggctggtttattgctgataaatctggagccggtgagcgtgggtctcgcggtatcattgcagcactggggccagatggtaagccctcccgtatcgtagttatctacacgacggggagtcaggcaactatggatgaacgaaatagacagatcgctgagataggtgcctcactgattaagcattggtaaccgattctaggtgcattggcgcagaaaaaaatgcctgatgcgacgctgcgcgtcttatactcccacatatgccagattcagcaacggatacggcttccccaacttgcccacttccatacgtgtcctccttaccagaaatttatccttaagatcccgaatcgtttaaactcgactctggctctatcgaatctccgtcgtttcgagcttacgcgaacagccgtggcgctcatttgctcgtcgggcatcgaatctcgtcagctatcgtcagcttacctttttggcagcgatcgcggctcccgacatcttggaccattagctccacaggtatcttcttccctctagtggtcataacagcagcttcagctacctctcaattcaaaaaacccctcaagacccgtttagaggccccaaggggttatgctatcaatcgttgcgttacacacacaaaaaaccaacacacatccatcttcgatggatagcgattttattatctaactgctgatcgagtgtagccagatctagtaatcaattacggggtcattagttcatagcccatatatggagttccgcgttacataacttacggtaaatggcccgcctggctgaccgcccaacgacccccgcccattgacgtcaataatgacgtatgttcccatagtaacgccaatagggactttccattgacgtcaatgggtggagtatttacggtaaactgcccacttggcagtacatcaagtgtatcatatgccaagtacgccccctattgacgtcaatgacggtaaatggcccgcctggcattatgcccagtacatgaccttatgggactttcctacttggcagtacatctacgtattagtcatcgctattaccatgctgatgcggttttggcagtacatcaatgggcgtggatagcggtttgactcacggggatttccaagtctccaccccattgacgtcaatgggagtttgttttggcaccaaaatcaacgggactttccaaaatgtcgtaacaactccgccccattgacgcaaatgggcggtaggcgtgtacggtgggaggtctatataagcagagctggtttagtgaaccgtcagatcagatctttgtcgatcctaccatccactcgacacacccgccagcggccgc

SEQ ID NO: 7 - DNA, 5148 bp, synthetic construct
  source 1..5148: mol_type = other DNA
gccaccatgtatccgtatgacgtcccggactatgcaggatcctatccatatgacgttccagattacgctatggtcttcacactcgaagatttcgttggggactggcgacagacagccggctacaacctggaccaagtccttgaacagggaggtgtgtccagtttgtttcagaatctcggggtgtccgtaactccgatccaaaggattgtcctgagcggtgaaaatgggctgaagatcgacatccatgtcatcatcccgtatgaaggtctgagcggcgaccaaatgggccagatcgaaaaaatttttaaggtggtgtaccctgtggatgatcatcactttaaggtgatcctgcactatggcacactggtaatcgacggggttacgccgaacatgatcgactatttcggacggccgtatgaaggcatcgccgtgttcgacggcaaaaagatcactgtaacagggaccctgtggaacggcaacaaaattatcgacgagcgcctgatcaaccccgacggctccctgctgttccgagtaaccatcaacggagtgaccggctggcggctgtgcgaacgcattctggcgggcggaggcggttctggtggcggaggttctgggggtggcggatctgcggcagcgatggatgtggataccccgagcggcaccaacagcggcgcgggcaagaagcgctttgaagtgaaaaagtggaatgcagtagccctctgggcctgggatattgtggttgataactgtgccatctgcaggaaccacattatggatctttgcatagaatgtcaagctaaccaggcgtccgctacttcagaagagtgtactgtcgcatggggagtctgtaaccatgcttttcacttccactgcatctctcgctggctcaaaacacgacaggtgtgtccattggacaacagagagtgggaattccaaaagtatgggcactagggatccgcaggcctctgctagcttgactgactgagatacagcgtaccttcagctcacagacatgataagatacattgatgagtttggacaaaccacaactagaatgcagtgaaaaaaatgctttatttgtgaaatttgtgatgctattgctttatttgtaaccattataagctgcaataaacaagttaacaacaacaattgcattcattttatgtttcaggttcagggggaggtgtgggaggttttttaaagcaagtaaaacctctacaaatgtggtattggcccatctctatcggtatcgtagcataaccccttggggcctctaaacgggtcttgaggggttttttgtgcccctcgggccggattgctatctaccggcattggcgcagaaaaaaatgcctgatgcgacgctgcgcgtcttatactcccacatatgccagattcagcaacggatacggcttccccaacttgcccacttccatacgtgtcctccttaccagaaatttatccttaaggtcgtcagctatcctgcaggcgatctctcgatttcgatcaagacattcctttaatggtcttttctggacaccactaggggtcagaagtagttcatcaaactttcttccctccctaatctcattggttaccttgggctatcgaaacttaattaaccagtcaagtcagctacttggcgagatcgacttgtctgggtttcgactacgctcagaattgcgtcagtcaagttcgatctggtccttgctattgcacccgttctccgattacgagtttcatttaaatcatgtgagcaaaaggccagcaaaaggccaggaaccgtaaaaaggccgcgttgctggcgtttttccataggctccgcccccctgacgagcatcacaaaaatcgacgctcaagtcagaggtggcgaaacccgacaggactataaagataccaggcgtttccccctggaagctccctcgtgcgctctcctgttccgaccctgccgcttaccggatacctgtccgcctttctcccttcgggaagcgtggcgctttctcatagctcacgctgtaggtatctcagttcggtgtaggtcgttcgctccaagctgggctgtgtgcacgaaccccccgttcagcccgaccgctgcgccttatccggtaactatcgtcttgagtccaacccggtaagacacgacttatcgccactggcagcagccactggtaacaggattagcagagcgaggtatgtaggcggtgctacagagttcttgaagtggtggcctaactacggctacactagaagaacagtatttggtatctgcgctctgctgaagccagttaccttcggaaaaagagttggtagctcttgatccggcaaacaaaccaccgctggtagcggtggtttttttgtttgcaagcagcagattacgcgcagaaaaaaaggatctcaagaagatcctttgatcttttctacggggtctgacgctcagtggaacgaaaactcacgttaagggattttggtcatgagattatcaaaaaggatcttcacctagatccttttaaattaaaaatgaagttttaaatcaatctaaagtatatatgagtaaacttggtctgacagttaccaatgcttaatcagtgaggcacctatctcagcgatctgtctatttcgttcatccatagttgcatttaaatttccgaactctccaaggccctcgtcggaaaatcttcaaacctttcgtccgatccatcttgcaggctacctctcgaacgaactatcgcaagtctcttggccggccttgcgccttggctattgcttggcagcgcctatcgccaggtattactccaatcccgaatatccgagatcgggatcacccgagagaagttcaacctacatcctcaatcccgatctatccgagatccgaggaatatcgaaatcggggcgcgcctggtgtaccgagaacgatcctctcagtgcgagtctcgacgatccatatcgttgcttggcagtcagccagtcggaatccagcttgggacccaggaagtccaatcgtcagatattgtactcaagcctggtcacggcagcgtaccgatctgtttaaacctagatattgatagtctgatcggtcaacgtataatcgagtcctagcttttgcaaacatctatcaagagacaggatcagcaggaggctttcgcatgagtattcaacatttccgtgtcgcccttattcccttttttgcggcattttgccttcctgtttttgctcacccagaaacgctggtgaaagtaaaagatgctgaagatcagttgggtgcgcgagtgggttacatcgaactggatctcaacagcggtaagatccttgagagttttcgccccgaagaacgctttccaatgatgagcacttttaaagttctgctatgtggcgcggtattatcccgtattgacgccgggcaagagcaactcggtcgccgcatacactattctcagaatgacttggttgagtattcaccagtcacagaaaagcatcttacggatggcatgacagtaagagaattatgcagtgctgccataaccatgagtgataacactgcggccaacttacttctgacaacgattggaggaccgaaggagctaaccgcttttttgcacaacatgggggatcatgtaactcgccttgatcgttgggaaccggagctgaatgaagccataccaaacgacgagcgtgacaccacgatgcctgtagcaatggcaacaaccttgcgtaaactattaactggcgaactacttactctagcttcccggcaacagttgatagactggatggaggcggataaagttgcaggaccacttctgcgctcggcccttccggctggctggtttattgctgataaatctggagccggtgagcgtgggtctcgcggtatcattgcagcactggggccagatggtaagccctcccgtatcgtagttatctacacgacggggagtcaggcaactatggatgaacgaaatagacagatcgctgagataggtgcctcactgattaagcattggtaaccgattctaggtgcattggcgcagaaaaaaatgcctgatgcgacgctgcgcgtcttatactcccacatatgccagattcagcaacggatacggcttccccaacttgcccacttccatacgtgtcctccttaccagaaatttatccttaagatcccgaatcgtttaaactcgactctggctctatcgaatctccgtcgtttcgagcttacgcgaacagccgtggcgctcatttgctcgtcgggcatcgaatctcgtcagctatcgtcagcttacctttttggcagcgatcgcggctcccgacatcttggaccattagctccacaggtatcttcttccctctagtggtcataacagcagcttcagctacctctcaattcaaaaaacccctcaagacccgtttagaggccccaaggggttatgctatcaatcgttgcgttacacacacaaaaaaccaacacacatccatcttcgatggatagcgattttattatctaactgctgatcgagtgtagccagatctagtaatcaattacggggtcattagttcatagcccatatatggagttccgcgttacataacttacggtaaatggcccgcctggctgaccgcccaacgacccccgcccattgacgtcaataatgacgtatgttcccatagtaacgccaatagggactttccattgacgtcaatgggtggagtatttacggtaaactgcccacttggcagtacatcaagtgtatcatatgccaagtacgccccctattgacgtcaatgacggtaaatggcccgcctggcattatgcccagtacatgaccttatgggactttcctacttggcagtacatctacgtattagtcatcgctattaccatgctgatgcggttttggcagtacatcaatgggcgtggatagcggtttgactcacggggatttccaagtctccaccccattgacgtcaatgggagtttgttttggcaccaaaatcaacgggactttccaaaatgtcgtaacaactccgccccattgacgcaaatgggcggtaggcgtgtacggtgggaggtctatataagcagagctggtttagtgaaccgtcagatcagatctttgtcgatcctaccatccactcgacacacccgccagcggccgc

SEQ ID NO: 8 - DNA, 5145 bp, synthetic construct
  source 1..5145: mol_type = other DNA
gccaccatggcggcagcgatggatgtggataccccgagcggcaccaacagcggcgcgggcaagaagcgctttgaagtgaaaaagtggaatgcagtagccctctgggcctgggatattgtggttgataactgtgccatctgcaggaaccacattatggatctttgcatagaatgtcaagctaaccaggcgtccgctacttcagaagagtgtactgtcgcatggggagtctgtaaccatgcttttcacttccactgcatctctcgctggctcaaaacacgacaggtgtgtccattggacaacagagagtgggaattccaaaagtatgggcacggcggaggcggttctggtggcggaggttctgggggtggcggatctgtcttcacactcgaagatttcgttggggactggcgacagacagccggctacaacctggaccaagtccttgaacagggaggtgtgtccagtttgtttcagaatctcggggtgtccgtaactccgatccaaaggattgtcctgagcggtgaaaatgggctgaagatcgacatccatgtcatcatcccgtatgaaggtctgagcggcgaccaaatgggccagatcgaaaaaatttttaaggtggtgtaccctgtggatgatcatcactttaaggtgatcctgcactatggcacactggtaatcgacggggttacgccgaacatgatcgactatttcggacggccgtatgaaggcatcgccgtgttcgacggcaaaaagatcactgtaacagggaccctgtggaacggcaacaaaattatcgacgagcgcctgatcaaccccgacggctccctgctgttccgagtaaccatcaacggagtgaccggctggcggctgtgcgaacgcattctggcgtatccgtatgacgtcccggactatgcaggatcctatccatatgacgttccagattacgcttaaggatccgcaggcctctgctagcttgactgactgagatacagcgtaccttcagctcacagacatgataagatacattgatgagtttggacaaaccacaactagaatgcagtgaaaaaaatgctttatttgtgaaatttgtgatgctattgctttatttgtaaccattataagctgcaataaacaagttaacaacaacaattgcattcattttatgtttcaggttcagggggaggtgtgggaggttttttaaagcaagtaaaacctctacaaatgtggtattggcccatctctatcggtatcgtagcataaccccttggggcctctaaacgggtcttgaggggttttttgtgcccctcgggccggattgctatctaccggcattggcgcagaaaaaaatgcctgatgcgacgctgcgcgtcttatactcccacatatgccagattcagcaacggatacggcttccccaacttgcccacttccatacgtgtcctccttaccagaaatttatccttaaggtcgtcagctatcctgcaggcgatctctcgatttcgatcaagacattcctttaatggtcttttctggacaccactaggggtcagaagtagttcatcaaactttcttccctccctaatctcattggttaccttgggctatcgaaacttaattaaccagtcaagtcagctacttggcgagatcgacttgtctgggtttcgactacgctcagaattgcgtcagtcaagttcgatctggtccttgctattgcacccgttctccgattacgagtttcatttaaatcatgtgagcaaaaggccagcaaaaggccaggaaccgtaaaaaggccgcgttgctggcgtttttccataggctccgcccccctgacgagcatcacaaaaatcgacgctcaagtcagaggtggcgaaacccgacaggactataaagataccaggcgtttccccctggaagctccctcgtgcgctctcctgttccgaccctgccgcttaccggatacctgtccgcctttctcccttcgggaagcgtggcgctttctcatagctcacgctgtaggtatctcagttcggtgtaggtcgttcgctccaagctgggctgtgtgcacgaaccccccgttcagcccgaccgctgcgccttatccggtaactatcgtcttgagtccaacccggtaagacacgacttatcgccactggcagcagccactggtaacaggattagcagagcgaggtatgtaggcggtgctacagagttcttgaagtggtggcctaactacggctacactagaagaacagtatttggtatctgcgctctgctgaagccagttaccttcggaaaaagagttggtagctcttgatccggcaaacaaaccaccgctggtagcggtggtttttttgtttgcaagcagcagattacgcgcagaaaaaaaggatctcaagaagatcctttgatcttttctacggggtctgacgctcagtggaacgaaaactcacgttaagggattttggtcatgagattatcaaaaaggatcttcacctagatccttttaaattaaaaatgaagttttaaatcaatctaaagtatatatgagtaaacttggtctgacagttaccaatgcttaatcagtgaggcacctatctcagcgatctgtctatttcgttcatccatagttgcatttaaatttccgaactctccaaggccctcgtcggaaaatcttcaaacctttcgtccgatccatcttgcaggctacctctcgaacgaactatcgcaagtctcttggccggccttgcgccttggctattgcttggcagcgcctatcgccaggtattactccaatcccgaatatccgagatcgggatcacccgagagaagttcaacctacatcctcaatcccgatctatccgagatccgaggaatatcgaaatcggggcgcgcctggtgtaccgagaacgatcctctcagtgcgagtctcgacgatccatatcgttgcttggcagtcagccagtcggaatccagcttgggacccaggaagtccaatcgtcagatattgtactcaagcctggtcacggcagcgtaccgatctgtttaaacctagatattgatagtctgatcggtcaacgtataatcgagtcctagcttttgcaaacatctatcaagagacaggatcagcaggaggctttcgcatgagtattcaacatttccgtgtcgcccttattcccttttttgcggcattttgccttcctgtttttgctcacccagaaacgctggtgaaagtaaaagatgctgaagatcagttgggtgcgcgagtgggttacatcgaactggatctcaacagcggtaagatccttgagagttttcgccccgaagaacgctttccaatgatgagcacttttaaagttctgctatgtggcgcggtattatcccgtattgacgccgggcaagagcaactcggtcgccgcatacactattctcagaatgacttggttgagtattcaccagtcacagaaaagcatcttacggatggcatgacagtaagagaattatgcagtgctgccataaccatgagtgataacactgcggccaacttacttctgacaacgattggaggaccgaaggagctaaccgcttttttgcacaacatgggggatcatgtaactcgccttgatcgttgggaaccggagctgaatgaagccataccaaacgacgagcgtgacaccacgatgcctgtagcaatggcaacaaccttgcgtaaactattaactggcgaactacttactctagcttcccggcaacagttgatagactggatggaggcggataaagttgcaggaccacttctgcgctcggcccttccggctggctggtttattgctgataaatctggagccggtgagcgtgggtctcgcggtatcattgcagcactggggccagatggtaagccctcccgtatcgtagttatctacacgacggggagtcaggcaactatggatgaacgaaatagacagatcgctgagataggtgcctcactgattaagcattggtaaccgattctaggtgcattggcgcagaaaaaaatgcctgatgcgacgctgcgcgtcttatactcccacatatgccagattcagcaacggatacggcttccccaacttgcccacttccatacgtgtcctccttaccagaaatttatccttaagatcccgaatcgtttaaactcgactctggctctatcgaatctccgtcgtttcgagcttacgcgaacagccgtggcgctcatttgctcgtcgggcatcgaatctcgtcagctatcgtcagcttacctttttggcagcgatcgcggctcccgacatcttggaccattagctccacaggtatcttcttccctctagtggtcataacagcagcttcagctacctctcaattcaaaaaacccctcaagacccgtttagaggccccaaggggttatgctatcaatcgttgcgttacacacacaaaaaaccaacacacatccatcttcgatggatagcgattttattatctaactgctgatcgagtgtagccagatctagtaatcaattacggggtcattagttcatagcccatatatggagttccgcgttacataacttacggtaaatggcccgcctggctgaccgcccaacgacccccgcccattgacgtcaataatgacgtatgttcccatagtaacgccaatagggactttccattgacgtcaatgggtggagtatttacggtaaactgcccacttggcagtacatcaagtgtatcatatgccaagtacgccccctattgacgtcaatgacggtaaatggcccgcctggcattatgcccagtacatgaccttatgggactttcctacttggcagtacatctacgtattagtcatcgctattaccatgctgatgcggttttggcagtacatcaatgggcgtggatagcggtttgactcacggggatttccaagtctccaccccattgacgtcaatgggagtttgttttggcaccaaaatcaacgggactttccaaaatgtcgtaacaactccgccccattgacgcaaatgggcggtaggcgtgtacggtgggaggtctatataagcagagctggtttagtgaaccgtcagatcagatctttgtcgatcctaccatccactcgacacacccgccagcggccgc

SEQ ID NO: 9 - DNA, 5553 bp, synthetic construct
  source 1..5553: mol_type = other DNA
gccaccatgtatccgtatgacgtcccggactatgcaggatcctatccatatgacgttccagattacgctgcagaaatcggtactggctttccattcgacccccattatgtggaagtcctgggcgagcgcatgcactacgtcgatgttggtccgcgcgatggcacccctgtgctgttcctgcacggtaacccgacctcctcctacgtgtggcgcaacatcatcccgcatgttgcaccgacccatcgctgcattgctccagacctgatcggtatgggcaaatccgacaaaccagacctgggttatttcttcgacgaccacgtccgcttcatggatgccttcatcgaagccctgggtctggaagaggtcgtcctggtcattcacgactggggctccgctctgggtttccactgggccaagcgcaatccagagcgcgtcaaaggtattgcatttatggagttcatccgccctatcccgacctgggacgaatggccagaatttgcccgcgagaccttccaggccttccgcaccaccgacgtcggccgcaagctgatcatcgatcagaacgtttttatcgagggtacgctgccgatgggtgtcgtccgcccgctgactgaagtcgagatggaccattaccgcgagccgttcctgaatcctgttgaccgcgagccactgtggcgcttcccaaacgagctgccaatcgccggtgagccagcgaacatcgtcgcgctggtcgaagaatacatggactggctgcaccagtcccctgtcccgaagctgctgttctggggcaccccaggcgttctgatcccaccggccgaagccgctcgcctggccaaaagcctgcctaactgcaaggctgtggacatcggcccgggtctgaatctgctgcaagaagacaacccggacctgatcggcagcgagatcgcgcgctggctgtcgacgctcgagatttccggcggcggaggcggttctagcaccaaccccccgcccccagagacctccaaccctaacaagcccaagaggcagaccaaccaactgcaatacctgctcagagtggtgctcaagacactatggaaacaccagtttgcatggcctttccagcagcctgtggatgccgtcaagctgaacctccctgattactataagatcattaaaacgcctatggatatgggaacaataaagaagcgcttggaaaacaactattactggaatgctcaggaatgtatccaggacttcaacactatgtttacaaattgttacatctacaacaagcctggagatgacatagtcttaatggcagaagctctggaaaagctcttcttgcaaaaaataaatgagctacccacagaagaatgaggatccgcaggcctctgctagcttgactgactgagatacagcgtaccttcagctcacagacatgataagatacattgatgagtttggacaaaccacaactagaatgcagtgaaaaaaatgctttatttgtgaaatttgtgatgctattgctttatttgtaaccattataagctgcaataaacaagttaacaacaacaattgcattcattttatgtttcaggttcagggggaggtgtgggaggttttttaaagcaagtaaaacctctacaaatgtggtattggcccatctctatcggtatcgtagcataaccccttggggcctctaaacgggtcttgaggggttttttgtgcccctcgggccggattgctatctaccggcattggcgcagaaaaaaatgcctgatgcgacgctgcgcgtcttatactcccacatatgccagattcagcaacggatacggcttccccaacttgcccacttccatacgtgtcctccttaccagaaatttatccttaaggtcgtcagctatcctgcaggcgatctctcgatttcgatcaagacattcctttaatggtcttttctggacaccactaggggtcagaagtagttcatcaaactttcttccctccctaatctcattggttaccttgggctatcgaaacttaattaaccagtcaagtcagctacttggcgagatcgacttgtctgggtttcgactacgctcagaattgcgtcagtcaagttcgatctggtccttgctattgcacccgttctccgattacgagtttcatttaaatcatgtgagcaaaaggccagcaaaaggccaggaaccgtaaaaaggccgcgttgctggcgtttttccataggctccgcccccctgacgagcatcacaaaaatcgacgctcaagtcagaggtggcgaaacccgacaggactataaagataccaggcgtttccccctggaagctccctcgtgcgctctcctgttccgaccctgccgcttaccggatacctgtccgcctttctcccttcgggaagcgtggcgctttctcatagctcacgctgtaggtatctcagttcggtgtaggtcgttcgctccaagctgggctgtgtgcacgaaccccccgttcagcccgaccgctgcgccttatccggtaactatcgtcttgagtccaacccggtaagacacgacttatcgccactggcagcagccactggtaacaggattagcagagcgaggtatgtaggcggtgctacagagttcttgaagtggtggcctaactacggctacactagaagaacagtatttggtatctgcgctctgctgaagccagttaccttcggaaaaagagttggtagctcttgatccggcaaacaaaccaccgctggtagcggtggtttttttgtttgcaagcagcagattacgcgcagaaaaaaaggatctcaagaagatcctttgatcttttctacggggtctgacgctcagtggaacgaaaactcacgttaagggattttggtcatgagattatcaaaaaggatcttcacctagatccttttaaattaaaaatgaagttttaaatcaatctaaagtatatatgagtaaacttggtctgacagttaccaatgcttaatcagtgaggcacctatctcagcgatctgtctatttcgttcatccatagttgcatttaaatttccgaactctccaaggccctcgtcggaaaatcttcaaacctttcgtccgatccatcttgcaggctacctctcgaacgaactatcgcaagtctcttggccggccttgcgccttggctattgcttggcagcgcctatcgccaggtattactccaatcccgaatatccgagatcgggatcacccgagagaagttcaacctacatcctcaatcccgatctatccgagatccgaggaatatcgaaatcggggcgcgcctggtgtaccgagaacgatcctctcagtgcgagtctcgacgatccatatcgttgcttggcagtcagccagtcggaatccagcttgggacccaggaagtccaatcgtcagatattgtactcaagcctggtcacggcagcgtaccgatctgtttaaacctagatattgatagtctgatcggtcaacgtataatcgagtcctagcttttgcaaacatctatcaagagacaggatcagcaggaggctttcgcatgagtattcaacatttccgtgtcgcccttattcccttttttgcggcattttgccttcctgtttttgctcacccagaaacgctggtgaaagtaaaagatgctgaagatcagttgggtgcgcgagtgggttacatcgaactggatctcaacagcggtaagatccttgagagttttcgccccgaagaacgctttccaatgatgagcacttttaaagttctgctatgtggcgcggtattatcccgtattgacgccgggcaagagcaactcggtcgccgcatacactattctcagaatgacttggttgagtattcaccagtcacagaaaagcatcttacggatggcatgacagtaagagaattatgcagtgctgccataaccatgagtgataacactgcggccaacttacttctgacaacgattggaggaccgaaggagctaaccgcttttttgcacaacatgggggatcatgtaactcgccttgatcgttgggaaccggagctgaatgaagccataccaaacgacgagcgtgacaccacgatgcctgtagcaatggcaacaaccttgcgtaaactattaactggcgaactacttactctagcttcccggcaacagttgatagactggatggaggcggataaagttgcaggaccacttctgcgctcggcccttccggctggctggtttattgctgataaatctggagccggtgagcgtgggtctcgcggtatcattgcagcactggggccagatggtaagccctcccgtatcgtagttatctacacgacggggagtcaggcaactatggatgaacgaaatagacagatcgctgagataggtgcctcactgattaagcattggtaaccgattctaggtgcattggcgcagaaaaaaatgcctgatgcgacgctgcgcgtcttatactcccacatatgccagattcagcaacggatacggcttccccaacttgcccacttccatacgtgtcctccttaccagaaatttatccttaagatcccgaatcgtttaaactcgactctggctctatcgaatctccgtcgtttcgagcttacgcgaacagccgtggcgctcatttgctcgtcgggcatcgaatctcgtcagctatcgtcagcttacctttttggcagcgatcgcggctcccgacatcttggaccattagctccacaggtatcttcttccctctagtggtcataacagcagcttcagctacctctcaattcaaaaaacccctcaagacccgtttagaggccccaaggggttatgctatcaatcgttgcgttacacacacaaaaaaccaacacacatccatcttcgatggatagcgattttattatctaactgctgatcgagtgtagccagatctagtaatcaattacggggtcattagttcatagcccatatatggagttccgcgttacataacttacggtaaatggcccgcctggctgaccgcccaacgacccccgcccattgacgtcaataatgacgtatgttcccatagtaacgccaatagggactttccattgacgtcaatgggtggagtatttacggtaaactgcccacttggcagtacatcaagtgtatcatatgccaagtacgccccctattgacgtcaatgacggtaaatggcccgcctggcattatgcccagtacatgaccttatgggactttcctacttggcagtacatctacgtattagtcatcgctattaccatgctgatgcggttttggcagtacatcaatgggcgtggatagcggtttgactcacggggatttccaagtctccaccccattgacgtcaatgggagtttgttttggcaccaaaatcaacgggactttccaaaatgtcgtaacaactccgccccattgacgcaaatgggcggtaggcgtgtacggtgggaggtctatataagcagagctggtttagtgaaccgtcagatcagatctttgtcgatcctaccatccactcgacacacccgccagcggccgc

SEQ ID NO: 10 - DNA, 5178 bp, synthetic construct
  source 1..5178: mol_type = other DNA
gccaccatgtatccgtatgacgtcccggactatgcaggatcctatccatatgacgttccagattacgctatggtcttcacactcgaagatttcgttggggactggcgacagacagccggctacaacctggaccaagtccttgaacagggaggtgtgtccagtttgtttcagaatctcggggtgtccgtaactccgatccaaaggattgtcctgagcggtgaaaatgggctgaagatcgacatccatgtcatcatcccgtatgaaggtctgagcggcgaccaaatgggccagatcgaaaaaatttttaaggtggtgtaccctgtggatgatcatcactttaaggtgatcctgcactatggcacactggtaatcgacggggttacgccgaacatgatcgactatttcggacggccgtatgaaggcatcgccgtgttcgacggcaaaaagatcactgtaacagggaccctgtggaacggcaacaaaattatcgacgagcgcctgatcaaccccgacggctccctgctgttccgagtaaccatcaacggagtgaccggctggcggctgtgcgaacgcattctggcgggcggaggcggttctagcaccaaccccccgcccccagagacctccaaccctaacaagcccaagaggcagaccaaccaactgcaatacctgctcagagtggtgctcaagacactatggaaacaccagtttgcatggcctttccagcagcctgtggatgccgtcaagctgaacctccctgattactataagatcattaaaacgcctatggatatgggaacaataaagaagcgcttggaaaacaactattactggaatgctcaggaatgtatccaggacttcaacactatgtttacaaattgttacatctacaacaagcctggagatgacatagtcttaatggcagaagctctggaaaagctcttcttgcaaaaaataaatgagctacccacagaagaatgaggatccgcaggcctctgctagcttgactgactgagatacagcgtaccttcagctcacagacatgataagatacattgatgagtttggacaaaccacaactagaatgcagtgaaaaaaatgctttatttgtgaaatttgtgatgctattgctttatttgtaaccattataagctgcaataaacaagttaacaacaacaattgcattcattttatgtttcaggttcagggggaggtgtgggaggttttttaaagcaagtaaaacctctacaaatgtggtattggcccatctctatcggtatcgtagcataaccccttggggcctctaaacgggtcttgaggggttttttgtgcccctcgggccggattgctatctaccggcattggcgcagaaaaaaatgcctgatgcgacgctgcgcgtcttatactcccacatatgccagattcagcaacggatacggcttccccaacttgcccacttccatacgtgtcctccttaccagaaatttatccttaaggtcgtcagctatcctgcaggcgatctctcgatttcgatcaagacattcctttaatggtcttttctggacaccactaggggtcagaagtagttcatcaaactttcttccctccctaatctcattggttaccttgggctatcgaaacttaattaaccagtcaagtcagctacttggcgagatcgacttgtctgggtttcgactacgctcagaattgcgtcagtcaagttcgatctggtccttgctattgcacccgttctccgattacgagtttcatttaaatcatgtgagcaaaaggccagcaaaaggccaggaaccgtaaaaaggccgcgttgctggcgtttttccataggctccgcccccctgacgagcatcacaaaaatcgacgctcaagtcagaggtggcgaaacccgacaggactataaagataccaggcgtttccccctggaagctccctcgtgcgctctcctgttccgaccctgccgcttaccggatacctgtccgcctttctcccttcgggaagcgtggcgctttctcatagctcacgctgtaggtatctcagttcggtgtaggtcgttcgctccaagctgggctgtgtgcacgaaccccccgttcagcccgaccgctgcgccttatccggtaactatcgtcttgagtccaacccggtaagacacgacttatcgccactggcagcagccactggtaacaggattagcagagcgaggtatgtaggcggtgctacagagttcttgaagtggtggcctaactacggctacactagaagaacagtatttggtatctgcgctctgctgaagccagttaccttcggaaaaagagttggtagctcttgatccggcaaacaaaccaccgctggtagcggtggtttttttgtttgcaagcagcagattacgcgcagaaaaaaaggatctcaagaagatcctttgatcttttctacggggtctgacgctcagtggaacgaaaactcacgttaagggattttggtcatgagattatcaaaaaggatcttcacctagatccttttaaattaaaaatgaagttttaaatcaatctaaagtatatatgagtaaacttggtctgacagttaccaatgcttaatcagtgaggcacctatctcagcgatctgtctatttcgttcatccatagttgcatttaaatttccgaactctccaaggccctcgtcggaaaatcttcaaacctttcgtccgatccatcttgcaggctacctctcgaacgaactatcgcaagtctcttggccggccttgcgccttggctattgcttggcagcgcctatcgccaggtattactccaatcccgaatatccgagatcgggatcacccgagagaagttcaacctacatcctcaatcccgatctatccgagatccgaggaatatcgaaatcggggcgcgcctggtgtaccgagaacgatcctctcagtgcgagtctcgacgatccatatcgttgcttggcagtcagccagtcggaatccagcttgggacccaggaagtccaatcgtcagatattgtactcaagcctggtcacggcagcgtaccgatctgtttaaacctagatattgatagtctgatcggtcaacgtataatcgagtcctagcttttgcaaacatctatcaagagacaggatcagcaggaggctttcgcatgagtattcaacatttccgtgtcgcccttattcccttttttgcggcattttgccttcctgtttttgctcacccagaaacgctggtgaaagtaaaagatgctgaagatcagttgggtgcgcgagtgggttacatcgaactggatctcaacagcggtaagatccttgagagttttcgccccgaagaacgctttccaatgatgagcacttttaaagttctgctatgtggcgcggtattatcccgtattgacgccgggcaagagcaactcggtcgccgcatacactattctcagaatgacttggttgagtattcaccagtcacagaaaagcatcttacggatggcatgacagtaagagaattatgcagtgctgccataaccatgagtgataacactgcggccaacttacttctgacaacgattggaggaccgaaggagctaaccgcttttttgcacaacatgggggatcatgtaactcgccttgatcgttgggaaccggagctgaatgaagccataccaaacgacgagcgtgacaccacgatgcctgtagcaatggcaacaaccttgcgtaaactattaactggcgaactacttactctagcttcccggcaacagttgatagactggatggaggcggataaagttgcaggaccacttctgcgctcggcccttccggctggctggtttattgctgataaatctggagccggtgagcgtgggtctcgcggtatcattgcagcactggggccagatggtaagccctcccgtatcgtagttatctacacgacggggagtcaggcaactatggatgaacgaaatagacagatcgctgagataggtgcctcactgattaagcattggtaaccgattctaggtgcattggcgcagaaaaaaatgcctgatgcgacgctgcgcgtcttatactcccacatatgccagattcagcaacggatacggcttccccaacttgcccacttccatacgtgtcctccttaccagaaatttatccttaagatcccgaatcgtttaaactcgactctggctctatcgaatctccgtcgtttcgagcttacgcgaacagccgtggcgctcatttgctcgtcgggcatcgaatctcgtcagctatcgtcagcttacctttttggcagcgatcgcggctcccgacatcttggaccattagctccacaggtatcttcttccctctagtggtcataacagcagcttcagctacctctcaattcaaaaaacccctcaagacccgtttagaggccccaaggggttatgctatcaatcgttgcgttacacacacaaaaaaccaacacacatccatcttcgatggatagcgattttattatctaactgctgatcgagtgtagccagatctagtaatcaattacggggtcattagttcatagcccatatatggagttccgcgttacataacttacggtaaatggcccgcctggctgaccgcccaacgacccccgcccattgacgtcaataatgacgtatgttcccatagtaacgccaatagggactttccattgacgtcaatgggtggagtatttacggtaaactgcccacttggcagtacatcaagtgtatcatatgccaagtacgccccctattgacgtcaatgacggtaaatggcccgcctggcattatgcccagtacatgaccttatgggactttcctacttggcagtacatctacgtattagtcatcgctattaccatgctgatgcggttttggcagtacatcaatgggcgtggatagcggtttgactcacggggatttccaagtctccaccccattgacgtcaatgggagtttgttttggcaccaaaatcaacgggactttccaaaatgtcgtaacaactccgccccattgacgcaaatgggcggtaggcgtgtacggtgggaggtctatataagcagagctggtttagtgaaccgtcagatcagatctttgtcgatcctaccatccactcgacacacccgccagcggccgc

SEQ ID NO: 11 - DNA, 8855 bp, synthetic construct
  source 1..8855: mol_type = other DNA
tcaatattggccattagccatattattcattggttatatagcataaatcaatattggctattggccattgcatacgttgtatctatatcataatatgtacatttatattggctcatgtccaatatgaccgccatgttggcattgattattgactagttattaatagtaatcaattacggggtcattagttcatagcccatatatggagttccgcgttacataacttacggtaaatggcccgcctggctgaccgcccaacgacccccgcccattgacgtcaataatgacgtatgttcccatagtaacgccaatagggactttccattgacgtcaatgggtggagtatttacggtaaactgcccacttggcagtacatcaagtgtatcatatgccaagtccgccccctattgacgtcaatgacggtaaatggcccgcctggcattatgcccagtacatgaccttacgggactttcctacttggcagtacatctacgtattagtcatcgctattaccatggtgatgcggttttggcagtacaccaatgggcgtggatagcggtttgactcacggggatttccaagtctccaccccattgacgtcaatgggagtttgttttggcaccaaaatcaacgggactttccaaaatgtcgtaataaccccgccccgttgacgcaaatgggcggtaggcgtgtacggtgggaggtctatataagcagagctggtttagtgaaccgtcagatcactagaagctttattgcggtagtttatcacagttaaattgctaacgcagtcagtgcttctgacacaacagtctcgaacttaagctgcagaagttggtcgtgaggcactgggcaggtaagtatcaaggttacaagacaggtttaaggagaccaatagaaactgggcttgtcgagacagagaagactcttgcgtttctgataggcacctattggtcttactgacatccactttgcctttctctccacaggtgtccactcccagttcaattacagctcttaaggctagagtattaatacgactcactatagggctagcgctcaccatggtcttcacactcgaagatttcgttggggactggcgacagacagccggctacaacctggaccaagtccttgaacagggaggtgtgtccagtttgtttcagaatctcggggtgtccgtaactccgatccaaaggattgtcctgagcggtgaaaatgggctgaagatcgacatccatgtcatcatcccgtatgaaggtctgagcggcgaccaaatgggccagatcgaaaaaatttttaaggtggtgtaccctgtggatgatcatcactttaaggtgatcctgcactatggcacactggtaatcgacggggttacgccgaacatgatcgactatttcggacggccgtatgaaggcatcgccgtgttcgacggcaaaaagatcactgtaacagggaccctgtggaacggcaacaaaattatcgacgagcgcctgatcaaccccgacggctccctgctgttccgagtaaccatcaacggagtgaccggctggcggctgtgcgaacgcattctggcgggctcgagcggcgcgatcgccatgtctgcggagagcggccctgggacgagattgagaaatctgccagtaatgggggatggactagaaacttcccaaatgtctacaacacaggcccaggcccaaccccagccagccaacgcagccagcaccaaccccccgcccccagagacctccaaccctaacaagcccaagaggcagaccaaccaactgcaatacctgctcagagtggtgctcaagacactatggaaacaccagtttgcatggcctttccagcagcctgtggatgccgtcaagctgaacctccctgattactataagatcattaaaacgcctatggatatgggaacaataaagaagcgcttggaaaacaactattactggaatgctcaggaatgtatccaggacttcaacactatgtttacaaattgttacatctacaacaagcctggagatgacatagtcttaatggcagaagctctggaaaagctcttcttgcaaaaaataaatgagctacccacagaagaaaccgagatcatgatagtccaggcaaaaggaagaggacgtgggaggaaagaaacagggacagcaaaacctggcgtttccacggtaccaaacacaactcaagcatcgactcctccgcagacccagacccctcagccgaatcctcctcctgtgcaggccacgcctcaccccttccctgccgtcaccccggacctcatcgtccagacccctgtcatgacagtggtgcctccccagccactgcagacgcccccgccagtgcccccccagccacaacccccacccgctccagctccccagcccgtacagagccacccacccatcatcgcggccaccccacagcctgtgaagacaaagaagggagtgaagaggaaagcagacaccaccacccccaccaccattgaccccattcacgagccaccctcgctgcccccggagcccaagaccaccaagctgggccagcggcgggagagcagccggcctgtgaaacctccaaagaaggacgtgcccgactctcagcagcacccagcaccagagaagagcagcaaggtctcggagcagctcaagtgctgcagcggcatcctcaaggagatgtttgccaagaagcacgccgcctacgcctggcccttctacaagcctgtggacgtggaggcactgggcctacacgactactgtgacatcatcaagcaccccatggacatgagcacaatcaagtctaaactggaggcccgtgagtaccgtgatgctcaggagtttggtgctgacgtccgattgatgttctccaactgctataagtacaaccctcctgaccatgaggtggtggccatggcccgcaagctccaggatgtgttcgaaatgcgctttgccaagatgccggacgagcctgaggagccagtggtggccgtgtcctccccggcagtgccccctcccaccaaggttgtggccccgccctcatccagcgacagcagcagcgatagctcctcggacagtgacagttcgactgatgactctgaggaggagcgagcccagcggctggctgagctccaggagcagctcaaagccgtgcacgagcagcttgcagccctctctcagccccagcagaacaaaccaaagaaaaaggagaaagacaagaaggaaaagaaaaaagaaaagcacaaaaggaaagaggaagtggaagagaataaaaaaagcaaagccaaggaacctcctcctaaaaagacgaagaaaaataatagcagcaacagcaatgtgagcaagaaggagccagcgcccatgaagagcaagccccctcccacgtatgagtcggaggaagaggacaagtgcaagcctatgtcctatgaggagaagcggcagctcagcttggacatcaacaagctccccggcgagaagctgggccgcgtggtgcacatcatccagtcacgggagccctccctgaagaattccaaccccgacgagattgaaatcgactttgagaccctgaagccgtccacactgcgtgagctggagcgctatgtcacctcctgtttgcggaagaaaaggaaacctcaagctgagaaagttgatgtgattgccggctcctccaagatgaagggcttctcgtcctcagagtcggagagctccagtgagtccagctcctctgacagcgaagactccgaaacagagatggctccgaagtcaaaaaagaaggggcaccccgggagggagcagaagaagcaccatcatcaccaccatcagcagatgcagcaggccccggctcctgtgccccagcagccgcccccgcctccccagcagcccccaccgcctccacctccgcagcagcaacagcagccgccacccccgcctcccccaccctccatgccgcagcaggcagccccggcgatgaagtcctcgcccccacccttcattgccacccaggtgcccgtcctggagccccagctcccaggcagcgtctttgaccccatcggccacttcacccagcccatcctgcacctgccgcagcctgagctgccccctcacctgccccagccgcctgagcacagcactccaccccatctcaaccagcacgcagtggtctctcctccagctttgcacaacgcactaccccagcagccatcacggcccagcaaccgagccgctgccctgcctcccaagcccgcccggcccccagccgtgtcaccagccttgacccaaacacccctgctcccacagccccccatggcccaacccccccaagtgctgctggaggatgaagagccacctgccccacccctcacctccatgcagatgcagctgtacctgcagcagctgcagaaggtgcagccccctacgccgctactcccttccgtgaaggtgcagtcccagcccccaccccccctgccgcccccaccccacccctctgtgcagcagcagctgcagcagcagccgccaccacccccaccaccccagccccagcctccaccccagcagcagcatcagccccctccacggcccgtgcacttgcagcccatgcagttttccacccacatccaacagcccccgccaccccagggccagcagcccccccatccgcccccaggccagcagccacccccgccgcagcctgccaagcctcagcaagtcatccagcaccaccattcaccccggcaccacaagtcggacccctactcaaccggtcacctccgcgaagccccctccccgcttatgatacattccccccagatgtcacagttccagagcctgacccaccagtctccaccccagcaaaacgtccagcctaagaaacaggagctgcgtgctgcctccgtggtccagccccagcccctcgtggtggtgaaggaggagaagatccactcacccatcatccgcagcgagcccttcagcccctcgctgcggccggagccccccaagcacccggagagcatcaaggcccccgtccacctgccccagcggccggaaatgaagcctgtggatgtcgggaggcctgtgatccggcccccagagcagaacgcaccgccaccaggggcccctgacaaggacaaacagaaacaggagccgaagactccagttgcgcccaaaaaggacctgaaaatcaagaacatgggctcctgggccagcctagtgcagaagcatccgaccaccccctcctccacagccaagtcatccagcgacagcttcgagcagttccgccgcgccgctcgggagaaagaggagcgtgagaaggccctgaaggctcaggccgagcacgctgagaaggagaaggagcggctgcggcaggagcgcatgaggagccgagaggacgaggatgcgctggagcaggcccggcgggcccatgaggaggcacgtcggcgccaggagcagcagcagcagcagcgccaggagcaacagcagcagcagcaacagcaagcagctgcggtggctgccgccgccaccccacaggcccagagctcccagccccagtccatgctggaccagcagagggagttggcccggaagcgggagcaggagcgaagacgccgggaagccatggcagctaccattgacatgaatttccagagtgatctattgtcaatatttgaagaaaatcttttcgtttaaacgaattcgggctcggtacccggggatcctctagagtcgacctgcaggcatgcaagctgatccggctgctaacaaagcccgaaaggaagctgagttggctgctgccaccgctgagcaataactagcataaccccttggggcggccgcttcgagcagacatgataagatacattgatgagtttggacaaaccacaactagaatgcagtgaaaaaaatgctttatttgtgaaatttgtgatgctattgctttatttgtaaccattataagctgcaataaacaagttaacaacaacaattgcattcattttatgtttcaggttcagggggagatgtgggaggtttttttaagcaagtaaaacctctacaaatgtggtaaaatcgaattttaacaaaatattaacgcttacaatttcctgatgcggtattttctccttacgcatctgtgcggtatttcacaccgcatacgcggatctgcgcagcaccatggcctgaaataacctctgaaagaggaacttggttaggtaccttctgaggcggaaagaaccagctgtggaatgtgtgtcagttagggtgtggaaagtccccaggctccccagcaggcagaagtatgcaaagcatgcatctcaattagtcagcaaccaggtgtggaaagtccccaggctccccagcaggcagaagtatgcaaagcatgcatctcaattagtcagcaaccatagtcccgcccctaactccgcccatcccgcccctaactccgcccagttccgcccattctccgccccatggctgactaattttttttatttatgcagaggccgaggccgcctcggcctctgagctattccagaagtagtgaggaggcttttttggaggcctaggcttttgcaaaaagcttaattaactgttgacaattaatcatcggcatagtatatcggcatagtataatacgacaaggtgaggaactaaacccaggaggcagatcatgattgaacaagatggattgcacgcaggttctccggccgcttgggtggagaggctattcggctatgactgggcacaacagacaatcggctgctctgatgccgccgtgttccggctgtcagcgcaggggcgcccggttctttttgtcaagaccgacctgtccggtgccctgaatgaactgcaggacgaggcagcgcggctatcgtggctggccacgacgggcgttccttgcgcagctgtgctcgacgttgtcactgaagcgggaagggactggctgctattgggcgaagtgccggggcaggatctcctgtcatctcaccttgctcctgccgagaaagtatccatcatggctgatgcaatgcggcggctgcatacgcttgatccggctacctgcccattcgaccaccaagcgaaacatcgcatcgagcgagcacgtactcggatggaagccggtcttgtcgatcaggatgatctggacgaagagcatcaggggctcgcgccagccgaactgttcgccaggctcaaggcgcgcatgcccgacggcgaggatctcgtcgtgacccatggcgatgcctgcttgccgaatatcatggtggaaaatggccgcttttctggattcatcgactgtggccggctgggtgtggcggaccgctatcaggacatagcgttggctacccgtgatattgctgaagagcttggcggcgaatgggctgaccgcttcctcgtgctttacggtatcgccgctcccgattcgcagcgcatcgccttctatcgccttcttgacgagttcttctgagcgggactctggggttcgaaatgaccgaccaagcgacgcccaacctgccatcacgatggccgcaataaaatatctttattttcattacatctgtgtgttggttttttgtgtgaatcgatagcgataaggatcctctttgcgcttgcgttttcccttgtccagatagcccagtagctgacattcatccggggtcagcaccgtttctgcggactggctttctacccggtatcagctcactcaaaggcggtaatacggttatccacagaatcaggggataacgcaggaaagaacatgtgagcaaaaggccagcaaaaggccaggaaccgtaaaaaggccgcgttgctggcgtttttccataggctccgcccccctgacgagcatcacaaaaatcgacgctcaagtcagaggtggcgaaacccgacaggactataaagataccaggcgtttccccctggaagctccctcgtgcgctctcctgttccgaccctgccgcttaccggatacctgtccgcctttctcccttcgggaagcgtggcgctttctcatagctcacgctgtaggtatctcagttcggtgtaggtcgttcgctccaagctgggctgtgtgcacgaaccccccgttcagcccgaccgctgcgccttatccggtaactatcgtcttgagtccaacccggtaagacacgacttatcgccactggcagcagccactggtaacaggattagcagagcgaggtatgtaggcggtgctacagagttcttgaagtggtggcctaactacggctacactagaaggacagtatttggtatctgcgctctgctgaagccagttaccttcggaaaaagagttggtagctcttgatccggcaaacaaaccaccgctggtagcggtggtttttttgtttgcaagcagcagattacgcgcagaaaaaaaggatttcaagaagatcctttgatcttttctacggggtctgacgctcagtggaacgaaaactcacgttaagggattttggtcatgagattatcaaaaaggatcttcacctagatccttttatagtccggaaatacaggaacgcacgctggatggcccttcgctgggatggtgaaaccatgaaaaatggcagcttcagtggattaagtgggggtaatgtggcctgtaccctctggttgcataggtattcatacggttaaaatttatcaggcgcgattgcggcagtttttcgggtggtttgttgccatttttacctgtctgctgccgtgatcgcgctgaacgcgttttagcggtgcgtacaattaagggattatggtaaatccacttactgtctgccctcgtagccatcgagataaaccgcagtactccggccacgatgcgtccggcgtagaggatcgagatct

SEQ ID NO: 12 - DNA, 6505 bp, synthetic construct
  source 1..6505: mol_type = other DNA
cggcagtgaaaaaaatgctttatttgtgaaatttgtgatgctattgctttatttgtaaccattataagctgcaataaacaagttaacaacaacaattgcattcattttatgtttcaggttcagggggaggtgtgggaggttttttaaagcaagtaaaacctctacaaatgtggtatggctgattatgatccgcggccgcaatacgtcgacgttatcagctgacttcgtacgagagcctaggattatggcgcgccactagttattaatagtaatcaattacggggtcattagttcatagcccatatatggagttccgcgttacataacttacggtaaatggcccgcctggctgaccgcccaacgacccccgcccattgacgtcaataatgacgtatgttcccatagtaacgccaatagggactttccattgacgtcaatgggtggagtatttacggtaaactgcccacttggcagtacatcaagtgtatcatatgccaagtccgccccctattgacgtcaatgacggtaaatggcccgcctggcattatgcccagtacatgaccttacgggactttcctacttggcagtacatctacgtattagtcatcgctattaccatggtgatgcggttttggcagtacaccaatgggcgtggatagcggtttgactcacggggatttccaagtctccaccccattgacgtcaatgggagtttgttttggcaccaaaatcaacgggactttccaaaatgtcgtaataaccccgccccgttgacgcaaatgggcggtaggcgtgtacggtgggaggtctatataagcagagctggtttagtgaaccgtcagatcactagaagctttattgcggtagtttatcacagttaaattgctaacgcagtcagtgcttctgacacaacagtctcgaacttaagctgcagaagttggtcgtgaggcactgggcaggtaagtatcaaggttacaagacaggtttaaggagaccaatagaaactgggcttgtcgagacagagaagactcttgcgtttctgataggcacctattggtcttactgacatccactttgcctttctctccacaggtgtccactcccagttcaattacagctcttaaggctagagtattaatacgactcactatagggctagcaaagccaccatggcagaaatcggtactggctttccattcgacccccattatgtggaagtcctgggcgagcgcatgcactacgtcgatgttggtccgcgcgatggcacccctgtgctgttcctgcacggtaacccgacctcctcctacgtgtggcgcaacatcatcccgcatgttgcaccgacccatcgctgcattgctccagacctgatcggtatgggcaaatccgacaaaccagacctgggttatttcttcgacgaccacgtccgcttcatggatgccttcatcgaagccctgggtctggaagaggtcgtcctggtcattcacgactggggctccgctctgggtttccactgggccaagcgcaatccagagcgcgtcaaaggtattgcatttatggagttcatccgccctatcccgacctgggacgaatggccagaatttgcccgcgagaccttccaggccttccgcaccaccgacgtcggccgcaagctgatcatcgatcagaacgtttttatcgagggtacgctgccgatgggtgtcgtccgcccgctgactgaagtcgagatggaccattaccgcgagccgttcctgaatcctgttgaccgcgagccactgtggcgcttcccaaacgagctgccaatcgccggtgagccagcgaacatcgtcgcgctggtcgaagaatacatggactggctgcaccagtcccctgtcccgaagctgctgttctggggcaccccaggcgttctgatcccaccggccgaagccgctcgcctggccaaaagcctgcctaactgcaaggctgtggacatcggcccgggtctgaatctgctgcaagaagacaacccggacctgatcggcagcgagatcgcgcgctggctgtcgacgctcgagatttccggcgagccaaccactgaggatctgtactttcagagcgataacgcgatcgccatggccggcgaaggagatcagcaggacgctgcgcacaacatgggcaaccacctgccgctcctgcctgcagagagtgaggaagaagatgaaatggaagttgaagaccaggatagtaaagaagccaaaaaaccaaacatcataaattttgacaccagtctgccgacatcacatacatacctaggtgctgatatggaagaatttcatggcaggactttgcacgatgacgacagctgtcaggtgattccagttcttccacaagtgatgatgatcctgattcccggacagacattacctcttcagctttttcaccctcaagaagtcagtatggtgcggaatttaattcagaaagatagaacctttgctgttcttgcatacagcaatgtacaggaaagggaagcacagtttggaacaacagcagagatatatgcctatcgagaagaacaggattttggaattgagatagtgaaagtgaaagcaattggaagacaaaggttcaaagtccttgagctaagaacacagtcagatggaatccagcaagctaaagtgcaaattcttcccgaatgtgtgttgccttcaaccatgtctgcagttcaattagaatccctcaataagtgccagatatttccttcaaaacctgtctcaagagaagaccaatgttcatataaatggtggcagaaataccagaagagaaagtttcattgtgcaaatctaacttcatggcctcgctggctgtattccttatatgatgctgagaccttaatggacagaatcaagaaacagctacgtgaatgggatgaaaatctaaaagatgattctcttccttcaaatccaatagatttttcttacagagtagctgcttgtcttcctattgatgatgtattgagaattcagctccttaaaattggcagtgctatccagcgacttcgctgtgaattagacattatgaataaatgtacttccctttgctgtaaacaatgtcaagaaacagaaataacaaccaaaaatgaaatattcagtttatccttatgtgggccgatggcagcttatgtgaatcctcatggatatgtgcatgagacacttactgtgtataaggcttgcaacttgaatctgataggccggccttctacagaacacagctggtttcctgggtatgcctggactgttgcccagtgtaagatctgtgcaagccatattggatggaagtttacggccaccaaaaaagacatgtcacctcaaaaattttggggcttaacgcgatctgctctgttgcccacgatcccagacactgaagatgaaataagtccagacaaagtaatactttgcttggtttaaacgaattcgggctcggtacccggggatcctctagagtcgacctgcaggcatgcaagctgatttggctgctgccaccgctgagcaaggccgcttcgagcagacatgataagatacattgatgagtttggacaaaccacaactagaatgcagtgaaaaaaatgctttatttgtgaaatttgtgatgctattgctttatttgtaaccattataagctgcaataaacaagttaacaacaacaattgcattcattttatgtttcaggttcagggggagatgtgggaggtttttttaagcaagtaaaacctctacaaatgtggtaaaatcttaattaagaattctaatataacttcgtatagcatacattatacgaagttatggatccactgttgacaattaatcatcggcatagtatatcggcatagtataatacgacaaggtgaggaactaaacccaggaggcagatcatgattgaacaagatggattgcacgcaggttctccggccgcttgggtggagaggctattcggctatgactgggcacaacagacaatcggctgctctgatgccgccgtgttccggctgtcagcgcaggggcgcccggttctttttgtcaagaccgacctgtccggtgccctgaatgaactgcaggacgaggcagcgcggctatcgtggctggccacgacgggcgttccttgcgcagctgtgctcgacgttgtcactgaagcgggaagggactggctgctattgggcgaagtgccggggcaggatctcctgtcatctcaccttgctcctgccgagaaagtatccatcatggctgatgcaatgcggcggctgcatacgcttgatccggctacctgcccattcgaccaccaagcgaaacatcgcatcgagcgagcacgtactcggatggaagccggtcttgtcgatcaggatgatctggacgaagagcatcaggggctcgcgccagccgaactgttcgccaggctcaaggcgcgcatgcccgacggcgaggatctcgtcgtgacccatggcgatgcctgcttgccgaatatcatggtggaaaatggccgcttttctggattcatcgactgtggccggctgggtgtggcggaccgctatcaggacatagcgttggctacccgtgatattgctgaagagcttggcggcgaatgggctgaccgcttcctcgtgctttacggtatcgccgctcccgattcgcagcgcatcgccttctatcgccttcttgacgagttcttctgattcgaaatgaccgaccaagcgacgcccaaccggtatcagctcactcaaaggcggtaatacggttatccacagaatcaggggataacgcaggaaagaacatgtgagcaaaaggccagcaaaaggccaggaaccgtaaaaaggccgcgttgctggcgtttttccataggctccgcccccctgacgagcatcacaaaaatcgacgctcaagtcagaggtggcgaaacccgacaggactataaagataccaggcgtttccccctggaagctccctcgtgcgctctcctgttccgaccctgccgcttaccggatacctgtccgcctttctcccttcgggaagcgtggcgctttctcatagctcacgctgtaggtatctcagttcggtgtaggtcgttcgctccaagctgggctgtgtgcacgaaccccccgttcagcccgaccgctgcgccttatccggtaactatcgtcttgagtccaacccggtaagacacgacttatcgccactggcagcagccactggtaacaggattagcagagcgaggtatgtaggcggtgctacagagttcttgaagtggtggcctaactacggctacactagaaggacagtatttggtatctgcgctctgctgaagccagttaccttcggaaaaagagttggtagctcttgatccggcaaacaaaccaccgctggtagcggtggtttttttgtttgcaagcagcagattacgcgcagaaaaaaaggatttcaagaagatcctttgatcttttctacggggtctgacgctcagtggaacgaaaactcacgttaagggattttggtcatgagattatcaaaaaggatcttcacctagatccttttatagtccggaatcgtcacacaaaaaaccaacacacagatgtaatgaaaataaagatattttattgcggccatcgtgatggctagagtttagccctcccacacataaccagagggcagcaattcacgaatcccaactgccgtcggctgtccatcactgtccttcactatggctttgatcccaggatgcagatcgagaagcacctgtcggcaccgtccgcaggggctcaagatgcccctgttctcatttccgatcgcgacgatacaagtcaggttgccagctgccgcagcagcagcagtgcccagcaccacgagttctgcacaaggtcccccagtaaaatgatatacattgacaccagtgaagatgcggccgtcgctagagagagctgcgctggcgacgctgtagtcttcagagatggggatgctgttgattgtagccgttgctctttcaatgagggtggattcttcttgagacaaaggcttggccatggtggcgctagtgtcagaagaatcgagctttttgcaaaagcctaggcctccaaaaaagcctcctcactacttctggaatagctcagaggccgaggcggcctcggcctctgcataaataaaaaaaattagtcagccatggggcggagaatgggcggaactgggcggagttaggggcgggatgggcggagttaggggcgggactatggttgctgactaattgagatgcatgctttgcatacttctgcctgctggggagcctggggactttccacacctggttgctgactaattgagatgcatgctttgcatacttctgcctgctggggagcctggggactttccacaccctaactgacacacattccacagctggttctttccgcctcagaaggtacctaaccaagttcctctttcagaggttatttcaggccatggtgctgcgcaagacgcgttaattaagacgt

SEQ ID NO: 13 - protein, 5 aa, synthetic construct
GGGGS

SEQ ID NO: 14 - protein, 15 aa, synthetic construct
GGGGSGGGGSGGGGS

SEQ ID NO: 15 - protein, 297 aa, synthetic construct
MAEIGTGFPFDPHYVEVLGERMHYVDVGPRDGTPVLFLHGNPTSSYVWRNIIPHVAPTHRCIAPDLIGMGKSDKPDLGYFFDDHVRFMDAFIEALGLEEVVLVIHDWGSALGFHWAKRNPERVKGIAFMEFIRPIPTWDEWPEFARETFQAFRTTDVGRKLIIDQNVFIEGTLPMGVVRPLTEVEMDHYREPFLNPVDREPLWRFPNELPIAGEPANIVALVEEYMDWLHQSPVPKLLFWGTPGVLIPPAEAARLAKSLPNCKAVDIGPGLNLLQEDNPDLIGSEIARWLSTLEISG

SEQ ID NO: 16 - protein, 171 aa, synthetic construct
MVFTLEDFVGDWRQTAGYNLDQVLEQGGVSSLFQNLGVSVTPIQRIVLSGENGLKIDIHVIIPYEGLSGDQMGQIEKIFKVVYPVDDHHFKVILHYGTLVIDGVTPNMIDYFGRPYEGIAVFDGKKITVTGTLWNGNKIIDERLINPDGSLLFRVTINGVTGWRLCERILA

SEQ ID NO: 17 - protein, 108 aa, synthetic construct [sequence omitted]

SEQ ID NO: 18 - protein, 21 aa, synthetic construct
MYPYDVPDYAGSYPYDVPDYA

SEQ ID NO: 19 - protein, 127 aa, synthetic construct
STNPPPPETSNPNKPKRQTNQLQYLLRVVLKTLWKHQFAWPFQQPVDAVKLNLPDYYKIIKTPMDMGTIKKRLENNYYWNAQECIQDFNTMFTNCYIYNKPGDDIVLMAEALEKLFLQKINELPTEE

SEQ ID NO: 20 - protein, 1363 aa, Homo sapiens
MSAESGPGTRLRNLPVMGDGLETSQMSTTQAQAQPQPANAASTNPPPPETSNPNKPKRQTNQLQYLLRVVLKTLWKHQFAWPFQQPVDAVKLNLPDYYKIIKTPMDMGTIKKRLENNYYWNAQECIQDFNTMFTNCYIYNKPGDDIVLMAEALEKLFLQKINELPTEETEIMIVQAKGRGRGRKETGTAKPGVSTVPNTTQASTPPQTQTPQPNPPPVQATPHPFPAVTPDLIVQTPVMTVVPPQPLQTPPPVPPQPQPPPAPAPQPVQSHPPIIAATPQPVKTKKGVKRKADTTTPTTIDPIHEPPSLPPEPKTTKLGQRRESSRPVKPPKKDVPDSQQHPAPEKSSKVSEQLKCCSGILKEMFAKKHAAYAWPFYKPVDVEALGLHDYCDIIKHPMDMSTIKSKLEAREYRDAQEFGADVRLMFSNCYKYNPPDHEVVAMARKLQDVFEMRFAKMPDEPEEPVVAVSSPAVPPPTKVVAPPSSSDSSSDSSSDSDSSTDDSEEERAQRLAELQEQLKAVHEQLAALSQPQQNKPKKKEKDKKEKKKEKHKRKEEVEENKKSKAKEPPPKKTKKNNSSNSNVSKKEPAPMKSKPPPTYESEEEDKCKPMSYEEKRQLSLDINKLPGEKLGRVVHIIQSREPSLKNSNPDEIEIDFETLKPSTLRELERYVTSCLRKKRKPQAEKVDVIAGSSKMKGFSSSESESSSESSSSDSEDSETEMAPKSKKKGHPGREQKKHHHHHHQQMQQAPAPVPQQPPPPPQQPPPPPPPQQQQQPPPPPPPPSMPQQAAPAMKSSPPPFIATQVPVLEPQLPGSVFDPIGHFTQPILHLPQPELPPHLPQPPEHSTPPHLNQHAVVSPPALHNALPQQPSRPSNRAAALPPKPARPPAVSPALTQTPLLPQPPMAQPPQVLLEDEEPPAPPLTSMQMQLYLQQLQKVQPPTPLLPSVKVQSQPPPPLPPPPHPSVQQQLQQQPPPPPPPQPQPPPQQQHQPPPRPVHLQPMQFSTHIQQPPPPQGQQPPHPPPGQQPPPPQPAKPQQVIQHHHSPRHHKSDPYSTGHLREAPSPLMIHSPQMSQFQSLTHQSPPQQNVQPKKQELRAASVVQPQPLVVVKEEKIHSPIIRSEPFSPSLRPEPPKHPESIKAPVHLPQRPEMKPVDVGRPVIRPPEQNAPPPGAPDKDKQKQEPKTPVAPKKDLKIKNMGSWASLVQKHPTTPSSTAKSSSDSFEQFRRAAREKEEREKALKAQAEHAEKEKERLRQERMRSREDEDALEQARRAHEEARRRQEQQQQQRQEQQQQQQQQAAAVAAAATPQAQSSQPQSMLDQQRELARKREQERRRREAMAATIDMNFQSDLLSIFEENLFV

SEQ ID NO: 21 - protein, 443 aa, Homo sapiens
MAGEGDQQDAAHNMGNHLPLLPAESEEEDEMEVEDQDSKEAKKPNIINFDTSLPTSHTYLGADMEEFHGRTLHDDDSCQVIPVLPQVMMILIPGQTLPLQLFHPQEVSMVRNLIQKDRTFAVLAYSNVQEREAQFGTTAEIYAYREEQDFGIEIVKVKAIGRQRFKVLELRTQSDGIQQAKVQILPECVLPSTMSAVQLESLNKCQIFPSKPVSREDQCSYKWWQKYQKRKFHCANLTSWPRWLYSLYDAETLMDRIKKQLREWDENLKDDSLPSNPIDFSYRVAACLPIDDVLRIQLLKIGSAIQRLRCELDIMNKCTSLCCKQCQETEITTKNEIFSLSLCGPMAAYVNPHGYVHETLTVYKACNLNLIGRPSTEHSWFPGYAWTVAQCKICASHIGWKFTATKKDMSPQKFWGLTRSALLPTIPDTEDEISPDKVILCLV

SEQ ID NO: 22 - protein, 580 aa, Homo sapiens
MKENKENSSPSVTSANLDHTKPCWYWDKKDLAHTPSQLEGLDPATEARYRREGARFIFDVGTRLGLHYDTLATGIIYFHRFYMFHSFKQFPRYVTGACCLFLAGKVEETPKKCKDIIKTARSLLNDVQFGQFGDDPKEEVMVLERILLQTIKFDLQVEHPYQFLLKYAKQLKGDKNKIQKLVQMAWTFVNDSLCTTLSLQWEPEIIAVAVMYLAGRLCKFEIQEWTSKPMYRRWWEQFVQDVPVDVLEDICHQILDLYSQGKQQMPHHTPHQLQQPPSLQPTPQVPQVQQSQPSQSSEPSQPQQKDPQQPAQQQQPAQQPKKPSPQPSSPRQVKRAVVVSPKEENKAAEPPPPKIPKIETTHPPLPPAHPPPDRKPPLAAALGEAEPPGPVDATDLPKVQIPPPAHPAPVHQPPPLPHRPPPPPPSSYMTGMSTTSSYMSGEGYQSLQSMMKTEGPSYGALPPAYGPPAHLPYHPHVYPPNPPPPPVPPPPASFPPPAIPPPTPGYPPPPPTYNPNFPPPPPRLPPTHAVPPHPPPGLGLPPASYPPPAVPPGGQPPVPPPIPPPGMPPVGGLGRAAWMR

SEQ ID NO: 23 - RNA, 20 nt, synthetic construct
  source 1..20: mol_type = other RNA
aagcctacttcaataaatga

SEQ ID NO: 24 - protein, 298 aa, Homo sapiens
MENFQKVEKIGEGTYGVVYKARNKLTGEVVALKKIRLDTETEGVPSTAIREISLLKELNHPNIVKLLDVIHTENKLYLVFEFLHQDLKKFMDASALTGIPLPLIKSYLFQLLQGLAFCHSHRVLHRDLKPQNLLINTEGAIKLADFGLARAFGVPVRTYTHEVVTLWYRAPEILLGCKYYSTAVDIWSLGCIFAEMVTRRALFPGDSEIDQLFRIFRTLGTPDEVVWPGVTSMPDYKPSFPKWARQDFSKVVPPLDEDGRSLLSQMLHYDPNKRISAKAALAHPFFQDVTKPVPHLRL

SEQ ID NO: 25 - protein, 22 aa, synthetic construct
GGGGSGGGGSYRSTSLYKKAGL

SEQ ID NO: 26 - protein, 20 aa, synthetic construct
DPAFLYKVVSGGGGSGGGGS

SEQ ID NO: 27 - protein, 626 aa, synthetic construct
MAPGQSKKKIFKPEELRQALMPTLEALYRQDPESLPFRQPVDPQLLGIPDYFDIVKSPMDLSTIKRKLDTGQYQEPWQYVDDIWLMFNNAWLYNRKTSRVYKYCSKLSEVFEQEIDPVMQSLGYCCGRKLEFSPQTLCCYGKQLCTIPRDATYYSYQNRYHFCEKCFNEIQGESVSLGDDPSQPQTTINKEQFSKRKNDTLDPELFVECTECGRKMHQICVLHHEIIWPAGFVCDGCLKKSARTRKENKFSAKRLPSTRLGTFLENRVNDFLRRQNHPESGEVTVRVVHASDKTVEVKPGMKARFVDSGEMAESFPYRTKALFAFEEIDGVDLCFFGMHVQEYGSDCPPPNQRRVYISYLDSVHFFRPKCLRTAVYHEILIGYLEYVKKLGYTTGHIWACPPSEGDDYIFHCHPPDQKIPKPKRLQEWYKKMLDKAVSERIVHDYKDIFKQATEDRLTSAKELPYFEGDFWPNVLEESIKELEQEEEERKREENTSNESTDVTKGDSKNAKKKNNKKTSKNKSSLSRGNKKKPGMPNVSNDLSQKLYATMEKHKEVFFVIRLIAGPAANSLPPIVDPDPLIPCDLMDGRDAFLTLARDKHLEFSSLRRAQWSTMCMLVELHTQSQD

SEQ ID NO: 28 - protein, 10 aa, synthetic construct
GGGGSGGGGS

SEQ ID NO: 29 - protein, 5 aa, synthetic construct
EAAAK

SEQ ID NO: 30 - protein, 10 aa, synthetic construct
EAAAKEAAAK

SEQ ID NO: 31 - protein, 15 aa, synthetic construct
EAAAKEAAAKEAAAK

SEQ ID NO: 32 - protein, 7 aa, synthetic construct
DYKDDDK

SEQ ID NO: 33 - protein, 14 aa, synthetic construct
DYKDDDKDYKDDDK

SEQ ID NO: 34 - protein, 21 aa, synthetic construct
DYKDDDKDYKDDDKDYKDDDK

SEQ ID NO: 35 - protein, 14 aa, synthetic construct
GKPIPNPLLGLDST

SEQ ID NO: 36 - protein, 28 aa, synthetic construct
GKPIPNPLLGLDSTGKPIPNPLLGLDST

SEQ ID NO: 37 - protein, 11 aa, synthetic construct
VSGWRLFKKIS

SEQ ID NO: 38 - protein, 11 aa, synthetic construct
VTGYRLFEEIL

SEQ ID NO: 39 - protein, 159 aa, synthetic construct
MVFTLEDFVGDWEQTAAYNLDQVLEQGGVSSLLQNLAVSVTPIQRIVRSGENALKIDIHVIIPYEGLSADQMAQIEEVFKVVYPVDDHHFKVILPYGTLVIDGVTPNMLNYFGRPYEGIAVFDGKKITVTGTLWNGNKIIDERLITPDGSMLFRVTINS

SEQ ID NO: 40 - protein, 214 aa, synthetic construct
MSKGEELFTGVVPILVELDGDVNGHKFSVRGEGEGDATIGKLTLKFICTTGKLPVPWPTLVTTLTYGVQCFSRYPDHMKRHDFFKSAMPEGYVQERTISFKDDGKYKTRAVVKFEGDTLVNRIELKGTDFKEDGNILGHKLEYNFNSHNVYITADKQKNGIKANFTVRHNVEDGSVQLADHYQQNTPIGDGPVLLPDNHYLSTQTVLSKDPNEK

SEQ ID NO: 41 - protein, 142 aa, synthetic construct
RDHMVLHEYVNAAGITGGSGGRDHMVLHEYVNAAGITGGSGGRDHMVLHEYVNAAGITGGSGGRDHMVLHEYVNAAGITGGSGGRDHMVLHEYVNAAGITGGSGGRDHMVLHEYVNAAGITGGSGGRDHMVLHEYVNAAGIT

SEQ ID NO: 42 - protein, 208 aa, synthetic construct
MEEDNMAIIKEFMRFKVHMEGSVNGHEFEIEGEGEGHPYEGTQTARLKVTKGDPLPFAWDILSPQFMYGSKAYVKHPADIPDYLKLSFPEGFTWERVMNFEDGGVVAVTQDSSLQDGQFIYKVKLLGINFPSDGPVMQKKTMGWEASTERMYPEDGALKGEINQRLKLKDGGHYDAEVKTTYRAKKPVQLPGAYDVDIKLDITSHNED

SEQ ID NO: 43 - protein, 16 aa, synthetic construct
YTIVEQYERAEARHST

SEQ ID NO: 44 - protein, 81 aa, Homo sapiens
MLIKVKTLTGKEIEIDIEPTDKVERIKERVEEKEGIPPQQQRLIYSGKQMNDEKTAADYKILGGSVLHLVLALRGGGGLRQ